European Patent Application EP 4 338 586 A2, published March 20, 2024. Title: ELITE EVENT CANOLA NS-B50027-4. Applicant: Nuseed Nutritional Australia Pty Ltd. Application WO PCT/US2017/038047, filed June 16, 2017. The sequence listing filed with the application follows.

SEQUENCE LISTING (66 sequences)

SEQ ID NO: 1 - DNA, 44 bp, synthetic construct
  misc_feature 1..44: note = KASP primer
  source 1..44: mol_type = other DNA
gaaggtgaccaagttcatgctccaagcaccgtagtaagagagca

SEQ ID NO: 2 - DNA, 26 bp, synthetic construct
  misc_feature 1..26: note = KASP primer
  source 1..26: mol_type = other DNA
gctaagaagtggggactcaactacaa

SEQ ID NO: 3 - DNA, 41 bp, synthetic construct
  misc_feature 1..41: note = KASP primer
  source 1..41: mol_type = other DNA
gaaggtgaccaagttcatgctgctcttgctggaactcttgg

SEQ ID NO: 4 - DNA, 26 bp, synthetic construct
  misc_feature 1..26: note = KASP primer
  source 1..26: mol_type = other DNA
gggttagccacattgtaggtaacgta

SEQ ID NO: 5 - DNA, 44 bp, synthetic construct
  misc_feature 1..44: note = KASP primer
  source 1..44: mol_type = other DNA
gaaggtgaccaagttcatgcttaagagacaccctggtggaaaga

SEQ ID NO: 6 - DNA, 28 bp, synthetic construct
  misc_feature 1..28: note = KASP primer
  source 1..28: mol_type = other DNA
tagcatcagttccaacttggtaagcaat

SEQ ID NO: 7 - DNA, 44 bp, synthetic construct
  misc_feature 1..44: note = KASP primer
  source 1..44: mol_type = other DNA
gaaggtgaccaagttcatgctgaacacgtaagcagaccaagcag

SEQ ID NO: 8 - DNA, 25 bp, synthetic construct
  misc_feature 1..25: note = KASP primer
  source 1..25: mol_type = other DNA
ccctcttctccctaacgaattcctt

SEQ ID NO: 9 - DNA, 44 bp, synthetic construct
  misc_feature 1..44: note = KASP primer
  source 1..44: mol_type = other DNA
gaaggtgaccaagttcatgctgaggaacctgttgctgctgatga

SEQ ID NO: 10 - DNA, 26 bp, synthetic construct
  misc_feature 1..26: note = KASP primer
  source 1..26: mol_type = other DNA
gcgatcctagcacaaagttgaaggta

SEQ ID NO: 11 - DNA, 44 bp, synthetic construct
  misc_feature 1..44: note = KASP primer
  source 1..44: mol_type = other DNA
gaaggtgaccaagttcatgctggatggatcgcttacctcttcgt

SEQ ID NO: 12 - DNA, 25 bp, synthetic construct
  misc_feature 1..25: note = KASP primer
  source 1..25: mol_type = other DNA
cagggtaaggttgtcctgtaacgtt

SEQ ID NO: 13 - DNA, 42 bp, synthetic construct
  misc_feature 1..42: note = KASP primer
  source 1..42: mol_type = other DNA
gaaggtgaccaagttcatgctctattggatggggactcaagc

SEQ ID NO: 14 - DNA, 26 bp, synthetic construct
  misc_feature 1..26: note = KASP primer
  source 1..26: mol_type = other DNA
gggagatccttagtagcagaagagat

SEQ ID NO: 15 - DNA, 44 bp, synthetic construct
  misc_feature 1..44: note = KASP primer
  source 1..44: mol_type = other DNA
gaaggtgaccaagttcatgctcctgagaggcgtcctgttgaaat

SEQ ID NO: 16 - DNA, 25 bp, synthetic construct
  misc_feature 1..25: note = KASP primer
  source 1..25: mol_type = other DNA
aacagcagccatatcagcagcagta

SEQ ID NO: 17 - DNA, 45 bp, synthetic construct
  misc_feature 1..45: note = KASP primer
  source 1..45: mol_type = other DNA
gaaggtgaccaagttcatgcttgttcttgggtgggtctgtccttc

SEQ ID NO: 18 - DNA, 46 bp, synthetic construct
  misc_feature 1..46: note = KASP primer
  source 1..46: mol_type = other DNA
gaaggtcggagtcaacggattgtgttcttgggtgggtctgtcctta

SEQ ID NO: 19 - DNA, 25 bp, synthetic construct
  misc_feature 1..25: note = KASP primer
  source 1..25: mol_type = other DNA
atccactagcagattgtcgtttccc

SEQ ID NO: 20 - DNA, 22 bp, synthetic construct
  misc_feature 1..22: note = KASP primer
  source 1..22: mol_type = other DNA
gttggctaaggtcacggtggag

SEQ ID NO: 21 - DNA, 48 bp, synthetic construct
  misc_feature 1..48: note = KASP primer
  source 1..48: mol_type = other DNA
gaaggtgaccaagttcatgctccgccttcagtttaaactatcagtgtt

SEQ ID NO: 22 - DNA, 41 bp, synthetic construct
  misc_feature 1..41: note = KASP primer
  source 1..41: mol_type = other DNA
gaaggtcggagtcaacggattggtcacggtggaggtcacca

SEQ ID NO: 23 - DNA, 22 bp, synthetic construct
  misc_feature 1..22: note = KASP primer
  source 1..22: mol_type = other DNA
ggtgtgttcttgggtgggtctg

SEQ ID NO: 24 - DNA, 49 bp, synthetic construct
  misc_feature 1..49: note = KASP primer
  source 1..49: mol_type = other DNA
gaaggtgaccaagttcatgctacttttttttcaactgttggctaaggta

SEQ ID NO: 25 - DNA, 49 bp, synthetic construct
  misc_feature 1..49: note = KASP primer
  source 1..49: mol_type = other DNA
gaaggtcggagtcaacggattacttttttttcaactgttggctaaggtc

SEQ ID NO: 26 - DNA, 21 bp, synthetic construct
  misc_feature 1..21: note = KASP primer
  source 1..21: mol_type = other DNA
gtgtgttcttgggtgggtctg

SEQ ID NO: 27 - DNA, 21 bp, synthetic construct
  misc_feature 1..21: note = KASP primer
  source 1..21: mol_type = other DNA
gtcgtttcccgccttcagttt

SEQ ID NO: 28 - DNA, 46 bp, synthetic construct
  misc_feature 1..46: note = KASP primer
  source 1..46: mol_type = other DNA
gaaggtgaccaagttcatgctaaactatcagtgtttgaacacctcc

SEQ ID NO: 29 - DNA, 44 bp, synthetic construct
  misc_feature 1..44: note = KASP primer
  source 1..44: mol_type = other DNA
gaaggtcggagtcaacggattacaacttgtcgtgctacacacct

SEQ ID NO: 30 - DNA, 22 bp, synthetic construct
  misc_feature 1..22: note = KASP primer
  source 1..22: mol_type = other DNA
ggttgtgtgaaaacgtgtgagc

SEQ ID NO: 31 - DNA, 51 bp, synthetic construct
  misc_feature 1..51: note = KASP primer
  source 1..51: mol_type = other DNA
gaaggtgaccaagttcatgctcttttagctaaataagaggttctgtatact

SEQ ID NO: 32 - DNA, 51 bp, synthetic construct
  misc_feature 1..51: note = KASP primer
  source 1..51: mol_type = other DNA
gaaggtcggagtcaacggattcttttagctaaataagaggttctgtataca

SEQ ID NO: 33 - DNA, 19 bp, synthetic construct
  misc_feature 1..19: note = KASP primer
  source 1..19: mol_type = other DNA
gattgtgattccgggcagt

SEQ ID NO: 34 - DNA, 21 bp, synthetic construct
  misc_feature 1..21: note = KASP primer
  source 1..21: mol_type = other DNA
gtgtgaaaacgtgtgagcaat

SEQ ID NO: 35 - DNA, 40 bp, synthetic construct
  misc_feature 1..40: note = KASP primer
  source 1..40: mol_type = other DNA
gaaggtgaccaagttcatgctttgtgattccgggcagtag

SEQ ID NO: 36 - DNA, 41 bp, synthetic construct
  misc_feature 1..41: note = KASP primer
  source 1..41: mol_type = other DNA
gaaggtcggagtcaacggatttgtgagcaattgttggaggt

SEQ ID NO: 37 - DNA, 31 bp, synthetic construct
  misc_feature 1..31: note = KASP primer
  source 1..31: mol_type = other DNA
tcttatcaacattaagaacataatcttttag

SEQ ID NO: 38 - DNA, 15 bp, synthetic construct
  misc_feature 1..15: note = Insertion deletion on Brassica chromosome A02
  source 1..15: mol_type = other DNA
gtagcacgacaagtt

SEQ ID NO: 39 - DNA, 20 bp, synthetic construct
  misc_feature 1..20: note = Insertion deletion Brassica chromosome A05
  source 1..20: mol_type = other DNA
cacggtggaggtcaccatgt

SEQ ID NO: 40 - DNA, 15004 bp, synthetic construct
  misc_feature 1..15004: note = Transgene insert and Brassica flanking regions
  source 1..15004: mol_type = other DNA
gagccttgagtgctactttgggaacaaaaacttggtttgatgctatcctagtctttttctcttttataaactattattagataaaaactaaaaaatagtatttatgagatttgtctttttttcacaatataaattattttaggtataaaaataaataatagaattagtattattagatatataaaatacatttaatttaattaataatataactgtaaagtataattaagttatacaatatctaataaatataaaaattgtattaaaatatgggaaaacaatattatattttaaagcgatcttactcgatctctctttgatcccaaagttttcattccttttaattatatttgttgcagaatattaaaaccagtgatttctggggtttgataggattaagacacgatcgcagagaaagtagaatcaatcgtggaagggaagggatattcgaaaccctaatttcgatcgtatccccatcttctacgaaagcatcgatcgacttttttctgattcagtgagagtttgaaatcaaagtttgattttttcgacctgatgggtttcttaaagaagttaacggggattttcgggttcgggcacaacgatggtgggcacggagctgctgcgagagacgaagatggtgaaggggataacactggatcagtctctgaggacggagataaacgccgggagggtaatcaggcaaggttccgtgaaaccggacttccaaggaggggttttggagttccggttcaagtagccgtcgaacggtctagtcctggtcctattcttcagccttgtgctgcttctgacggtggagttcaggtttgtctttctttcatggttgtgattttaactgtgtagaagtctagggactgaagaaattaatgagaatttgagggttgctagttttgattctgatcttgtaatgtggctacagtgttgtacttgtcttgttgcaggatcgttaaatccatttgtttggttccgatcatcctatgttagttggtaaaattggtcttgtgagtttgtttaagttgtttttgtgtcttcattcattttctaagcttagcattgatgaacagttgaatttagaatctttgttctaagcttaacattaatgaatatcgaatctttgttctactcagtcctttctttgtttttggttgtgatatgttctcgtttcaacgtagtttatgttcttcttgtgattggctttacattctgcacggtttccgctttagttaggtgtctgcattatagttagttcattgctatcttaaattctctgttcattcatctctatatatcaaattaaagagtggcagtgaagtttatgacaggacacgatatatgttttagcttgattagttgcggttaaagcaaaaagtttttgtttcactctgtctgctacagaacctgtaatttagaaatgatgatggatctcatgtcttaacggtttcgtattcatcatgagtcacgaggctgctatagagtttgaatcttaattggttctgttgttggggaaagacaataatccagtctttaagaagctagtggggttgattcatccccaagactattcgattgtccaaacgcattgatatgttttttttaatcaagtttttgttgatggcaataaactaacatcccagcatagttattgactcgacttagttttaccattagggactacgatggtactcaatgcggctaaggattgatgaagatggagatgttgcagatgagttcttggaagatgataactgtaagactttgcccagaaaatgcaaaacaaaagctgcaaaagtgagaggtttagtgatatcttctgatgggaaacttcagccattaatgcattgagcagtgaacaccaaggataaatatttactgattagtgtgtgattgaatcaaagaaaggttagaatctggttttcatttagccattcaatctcgatgtaaaatcggttagattctggttgttgatacttgagaacttgaaatgttttgtaactgtgaattttgttttgaaaatagacaagtgaatctgtttggggttgtgtgaaaacgtgtgagcaattgttggaggtgttcaaacactgatagtttaaactgaaggcgggaaacgacaatctgctagtggatctcccagtcacgacgttgtaaaacgggcgccccgcggaaagcttgcggccgcggtaccgcccgttcgactcagatcttccaaggcctcgtctccgagtccgctgcttctcgccgcgccgatcacttctccgccgccaacaaggcttgtagttaataggaatcattcagggattgtgattccgggcagtagtaattaataatatagtattagtatagataatatgtttcgtttgggatctttggaacgttgctctgttccttgttgttcattttaaagcttttgagggatagttgcagaactgttcggtgatgcttcatcctctcaagaactagatttgggtaaagaaacatccatgcatggatatggaatgttgttcttccgattggagattattttataaaatttaaaattcatgatttaaaaaaacacataaaaaccacaaaattcatgatttattgacaatacgatacaaaattagcaccaccggctactggctcattacacatttccccttcccctcattctcactttgtggctttattattattattattacatatattttaccgttattatttcacgtcacataagcttgttaattaatcattagtgagccttctcagcctttccgttaacgtagtagtgctgtcccaccttatcaaggttagagaaagtagccttccaagcaccgtagtaagagagcaccttgtagttgagtccccacttcttagcgaaaggaacgaatcttctgctaacctcaggctgtctgaattgaggcatatcagggaagaggtggtggataacctgacagttaaggtatcccataagccagttcacgtatcctctagaaggatcgatatcaacggtgtgatcaacagcgtagttaacccaagaaaggtgcttatcagatggaacaacagggaggtgagtatgagaagtagagaagtgagcgaaaaggtacatgtaagcgatccagtttccgaaagtgaaccaccagtaagcaacaggccaagagtatccagtagcaagcttgataacagcggttctaacaacatgagaaacgagcatccaagaagcctcttcgtagttcttcttacggagaacttgtctagggtggagaacgtagatccagaaagcttgaacaagaagtccagaggtaacaggaacgaaagtccaagcttgaagtctagcccaagctctagagaatcctctaggtctgttatcctcaacagcagtgttgaagaaagccacagcaggagtggtatcaagatccatatcgtgtctaaccttttgaggggtagcatggtgcttgttatgcatctggttccacatctcaccagaagtagaaagtccgaatccacaagtcatagcctgaagtctcttgtccacgtaaacagatccggtaagagagttatgtccaccctcatgttgaacccatccacatctagctccgaagaaagcaccgtaaacaacagaagcaatgatagggtatccagcgtacataagagcagttccaagagcgaatgtagcaagaagctcgagaagtctgtaagccacatgggtgatagaaggcttgaagaatccatctctctcaagctcagcacgccatctagcgaaatcctcaagcataggagcatcctcagactcagatctcttgatctcagcaggtctagaaggcaaagctctaagcatcttccaagccttgagagaacgcatgtggaattctttgaaagcctcagtagcatcagcaccagtgttagcaagcatgtagaagatcacagatccaccagggtgcttgaagttagtcacatcgtactcaacgtcctcaactctaacccatctagtctcgaaagtagcagcaagctcatgaggctcaagagtcttaagatcaacaggagcagtagaagcatccttagcatcaagagcctcagcagaagatttagacctggtaagtggagatctaggagaagatcttccatcagtcttaggagggcacatggtatggtaattgtaaatgtaattgtaatgttgtttgttgtttgttgttgttggtaattgttgtaaaattaattaagtgggtatcttttggatggataagcaagtagtgatgatgttctaggtgaagtgatgggggtgttttatagcgggagatggtgaaatggatggtcgccacataagaaatggaggggaagggttcttgcgccattcttcagtttgcatggatgcatgggtttcattttgtaacacgtaataaggacaatgaagtgcaggtgtctctcaagtttcagaggggatatgtggacagaagaagaacggcgatgatattgatggaaatggccatctagtgtgaatctattcggttgataatactagtgcattttggccgttaatcccttcaattaactgcacaaacttcagttgagtattgattatttgattataggttctgtaaacacaataccaagtttatttagaggggagacatacaaatagtttcgatataaataatagagtggttaaacttagttattaaaactatatataaagtctaaaagttaaattatttttttaattgcaaatatataaagtctaaaggggttacattatttcttaagagatgtaactctgttggaatctgacttaatccgtctcatcactctggtttccagttctaatctaatgaattgttttctgccaaagaatttgaagcaagaagtaaattgatcaatgccgtcaacccacaccaaaccgtcaacccactaccatcgccgcggagacccccaaactcaacctccacccatcggtaagaagcacagggcagcccgcaccaccaccaatttggcgtgcatgacacctagggacttggcacgggaggcggcgcacgtggatgcaaatgacgggatatcagatgacaggaaacgacgttgagagaccatacgatgtagaatatgagctcaccatcaacgagaaactaggaaaatcacaaaaaaaacaactctcgtaattgtacgagtggcacagatgggtctgcctcaacatatctctaatacggcgaagcctgcccaacacgtagttgccggaatccggtgtggagctcacgactctgaaagataggcgcttcctgtttcgtttcgctcacccactggacgtccgtcatgtgatggatttcggtcattggtttgctgacaaccacattctgaagctccatgagatgagtcttcacaataggtcctgctcaataccgtggagttatggttgcaagtccataacttgccgttcgaatattttgcggagccagtcggacgggaattggcgagctcggctgacacctataaaggccatgacaagaagaaccaaaagttcttccctaatgctttcatgaggcttcgggtcgttatggatgtcggaaaacccctcttgaaggaacgagacgttattatgcatgacggtaagactattacttgtcagtataagtatgaaagattacctgtcttctgctttgtttgtggattgattggacacgttgaaaaaaaatgtgcacttcgatttcaatactcagagatcgacttcccttttctctaggagtattcgatcaaggcattaacatggaaggaagctcaagctctaaaggcttcacaatggaacctgaaaaatttcaacaagcctaaactgaaatcgaagtcaaatcacccaaccgggagctctaaatcagcaaacactcctcctccacagtatccaatcatcgtgcacgatgctccaggtattgcaagccaggtattgcaagctaggagtaggatagagaccttaaacgtcgttggtgtgaagagtcatcttcagacctaatggagatagatgtagacggcggcacgaagactctgaaacaccagaaaggctagtccaggataaggatctgctatcccaactgacctctcgttagtcccaaggcctctcaactagagcaggaggaaggatggtcacaagactaggataatgatgtttccaatatgaacctgaatgtccatagctaatttttttagtcttgcttctgcactttttgtttattatgttctggtgactatgttatttacccttgtccgtatgcttgagggtaccctagtagattggttggttggtttccatgtaccagaaggcttaccctattagttgaaagttgaaactttgttccctactcaattcctagttgtgtaaatgtatgtatatgtaatgtgtataaaacgtagtacttaaatgactaggagtggttcttgagaccgatgagagatgggagcagaactaaagatgatgacataattaagaacgaatttgaaaggctcttaggtttgaatcctattcgagaatgtttttgtcaaagatagtggcgattttgaaccaaagaaaacatttaaaaaatcagtatccggttacgttcatgcaaatagaaagtggtctaggatctgattgtaattttagacttaaagagtctcttaagattcaatcctggctgtgtacaaaactacaaataatatattttagactatttggccttaactaaacttccactcattatttactgaggttagagaatagacttgcgaataaacacattcccgagaaatactcatgatcccataattagtcagagggtatgccaatcagatctaagaacacacattccctcaaattttaatgcacatgtaatcatagtttagcacaattcaaaaataatgtagtattaaagacagaaatttgtagacttttttttggcgttaaaagaagactaagtttatacgtacattttattttaagtggaaaaccgaaattttccatcgaaatatatgaatttagtatatatatttctgcaatgtactattttgctattttggcaactttcagtggactactactttattacaatgtgtatggatgcatgagtttgagtatacacatgtctaaatgcatgctttgtaaaacgtaacggaccacaaaagaggatccatacaaatacatctcatagcttcctccattattttccgacacaaacagagcattttacaacaattaccaacaacaacaaacaacaaacaacattacaattacatttacaattaccataccatggcctctatcgctatccctgctgctcttgctggaactcttggatacgttacctacaatgtggctaaccctgatatcccagcttctgagaaagttcctgcttacttcatgcaggttgagtactggggacctactatcggaactattggatacctcctcttcatctacttcggaaagcgtatcatgcagaacagatctcaacctttcggactcaagaacgctatgctcgtttacaacttctaccagaccttcttcaacagctactgcatctaccttttcgttacttctcatagggctcagggacttaaggtttggggaaacatccctgatatgactgctaactcttggggaatctctcaggttatctggcttcactacaacaacaagtacgttgagcttctcgacaccttcttcatggtgatgaggaagaagttcgaccagctttctttccttcacatctaccaccacactcttctcatctggtcatggttcgttgttatgaagcttgagcctgttggagattgctacttcggatcttctgttaacaccttcgtgcacgtgatcatgtactcttactacggacttgctgctcttggagttaactgtttctggaagaagtacatcacccagatccagatgcttcagttctgtatctgtgcttctcactctatctacaccgcttacgttcagaataccgctttctggcttccttaccttcaactctgggttatggtgaacatgttcgttctcttcgccaacttctaccgtaagaggtacaagtctaagggtgctaagaagcagtgataaggcgcgcggcgcgccgggccgccgccatgtgacagatcgaaggaagaaagtgtaataagacgactctcactactcgatcgctagtgattgtcattgttatatataataatgttatctttcacaacttatcgtaatgcatgtgaaactataacacattaatcctacttgtcatatgataacactctccccatttaaaactcttgtcaatttaaagatataagattctttaaatgattaaaaaaaatatattataaattcaatcactcctactaataaattattaattattatttattgattaaaaaaatacttatactaatttagtctgaatagaataattagattctagtctcatccccttttaaaccaacttagtaaacgtttttttttttaattttatgaagttaagtttttaccttgtttttaaaaagaatcgttcataagatgccatgccagaacattagctacacgttacacatagcatgcagccgcggagaattgtttttcttcgccacttgtcactcccttcaaacacctaagagcttctctctcacagcacacacatacaatcacatgcgtgcatgcattattacacgtgatcgccatgcaaatctcctttatagcctataaattaactcatccgcttcactctttactcaaaccaaaactcatcgatacaaacaagattaaaaacatacacgaggatcttttacaacaattaccaacaacaacaaacaacaaacaacattacaattacatttacaattaccataccatgcctccaagggactcttactcttatgctgctcctccttctgctcaacttcacgaagttgatactcctcaagagcacgacaagaaagagcttgttatcggagatagggcttacgatgttaccaacttcgttaagagacaccctggtggaaagatcattgcttaccaagttggaactgatgctaccgatgcttacaagcagttccatgttagatctgctaaggctgacaagatgcttaagtctcttccttctcgtcctgttcacaagggatactctccaagaagggctgatcttatcgctgatttccaagagttcaccaagcaacttgaggctgagggaatgttcgagccttctcttcctcatgttgcttacagacttgctgaggttatcgctatgcatgttgctggtgctgctcttatctggcatggatacactttcgctggaatcgctatgcttggagttgttcagggaagatgtggatggcttatgcatgagggtggacattactctctcactggaaacattgctttcgacagagctatccaagttgcttgttacggacttggatgtggaatgtctggtgcttggtggcgtaaccagcataacaagcaccatgctactcctcaaaagcttcagcacgatgttgatcttgatacccttcctctcgttgctttccatgagagaatcgctgctaaggttaagtctcctgctatgaaggcttggctttctatgcaagctaagcttttcgctcctgttaccactcttcttgttgctcttggatggcagctttaccttcatcctagacacatgctcaggactaagcactacgatgagcttgctatgctcggaatcagatacggacttgttggataccttgctgctaactacggtgctggatacgttctcgcttgttaccttctttacgttcagcttggagctatgtacatcttctgcaacttcgctgtttctcatactcacctccctgttgttgagcctaacgagcatgctacttgggttgagtacgctgctaaccacactactaactgttctccatcttggtggtgtgattggtggatgtcttaccttaactaccagatcgagcaccacctttacccttctatgcctcaattcagacaccctaagatcgctcctagagttaagcagcttttcgagaagcacggacttcactacgatgttagaggatacttcgaggctatggctgatactttcgctaaccttgataacgttgcccatgctcctgagaagaaaatgcagtaatgagatcgttcaaacatttggcaataaagtttcttaagattgaatcctgttgccggtcttgcgatgattatcatataatttctgttgaattacgttaagcacgtaataattaacatgtaatgcatgacgttatttatgagatgggtttttatgattagagtcccgcaattatacatttaatacgcgatagaaaacaaaatatagcgcgcaaactaggataaattatcgcgcgcggtgtcatctatgttactagatcggtcgattaaaaatcccaattatatttggtctaatttagtttggtattgagtaaaacaaattcgaaccaaaccaaaatataaatatatagtttttatatatatgcctttaagactttttatagaattttctttaaaaaatatctagaaatatttgcgactcttctggcatgtaatatttcgttaaatatgaagtgctccatttttattaactttaaataattggttgtacgatcactttcttatcaagtgttactaaaatgcgtcaatctctttgttcttccatattcatatgtcaaaatctatcaaaattcttatatatctttttcgaatttgaagtgaaatttcgataatttaaaattaaatagaacatatcattatttaggtatcatattgatttttatacttaattactaaatttggttaactttgaaagtgtacatcaacgaaaaattagtcaaacgactaaaataaataaatatcatgtgttattaagaaaattctcctataagaatattttaatagatcatatgtttgtaaaaaaaattaatttttactaacacatatatttacttatcaaaaatttgacaaagtaagattaaaataatattcatctaacaaaaaaaaaaccagaaaatgctgaaaacccggcaaaaccgaaccaatccaaaccgatatagttggtttggtttgattttgatataaaccgaaccaactcggtccatttgcacccctaatcataatagctttaatatttcaagatattattaagttaacgttgtcaatatcctggaaattttgcaaaatgaatcaagcctatatggctgtaatatgaatttaaaagcagctcgatgtggtggtaatatgtaatttacttgattctaaaaaaatatcccaagtattaataatttctgctaggaagaaggttagctacgatttacagcaaagccagaatacaaagaaccataaagtgattgaagctcgaaatatacgaaggaacaaatatttttaaaaaaatacgcaatgacttggaacaaaagaaagtgatatattttttgttcttaaacaagcatcccctctaaagaatggcagttttcctttgcatgtaactattatgctcccttcgttacaaaaattttggactactattgggaacttcttctgaaaatagtgatagaacccacacgagcatgtgctttccatttaattttaaaaaccaagaaacatacatacataacattccatcagcctctctctctttttattacggttaatgacttaaaacacatcttattatcccatccttaacacctagcagtgtctttatacgatctcatcgatcaccacttcaaaaccatgcagactgctgctgcccctggagctggcatcggctaggctgggtgccgcactgtcccggaaggtccctagcgacttgtttagattgatgggaccacctctcaacttcctgctgctgtccctgctgctggatgtcctgcctcatctggccgattgcacgctccagtcccctgcatgtgcactcgctcctcaattgcttaagatcatcgcagcagctatcgaagtgctggctctgttgccctcctccacggccttggttgtagtagtagctgccgccgcccttctggactttttcccacaggaaccgccgaataattcgatagaaccacacgagcatgtgctttcatttattttaaaaaccaagaaacatacataacatttcatcagcctctctctctctctctctctctctctctctctctctctctctctctctctctttattacagctgttacactaacttaaaacacattcatctcattattattattattatccatccttaacacctagcagtgtctttgtacgatctcataatcgatcaccccttcatcaggtatccttaggcttcactccaacgttgttgcagttacggaacatgtacacaccatcatggttctcaacgaactggcaagatctccaagttttccaaaggctaacccacatgttctcatcggtgtgtctgtagtgctctcccataactttcttgatgcactcggtagcttctctagcatggtagaatgggatccttgaaacgtagtgatggagcacatgagtctcgatgatgtcatggaagatgattccgaggattccgaactctctatcgatagtagcagcagcacccttagcgaaagtccactcttgagcatcgtaatgaggcatagaagaatcggtgtgctgaaggaaggtaacgaaaacaagccagtggttaacaaggatccaaggacagaaccatgtgatgaaagtaggccagaatccgaaaaccttgtaagcggtgtaaacagaagtgagggtagcaaggattccaagatcagaaagaacgatgtaccagtagtccttcttatcgaaaacagggctagaaggccagtagtgagacttgaagaacttagaaacaccagggtaaggttgtccagtagcgttagtagcaaggtaaagagaaagtcctccaagctgttggaacaagagagcgaaaacagagtagataggagtttcctcagcgatatcgtgaaggctggtaacttggtgcttctctttgaattcctcggcggtgtaaggaacgaaaaccatatctctggtcatgtgtccagtagccttatggtgcttagcatgagagaacttccagctgaagtaaggaaccataacaagagagtggagaacccatccaacggtatcgttaacccatccgtagttagagaaagcagaatgtccacactcatgtccaaggatccagattccgaatccgaaacaagagatagagaacacgtaagcagaccaagcagcgaatctaaggaattcgttagggagaagagggatgtaggtaagtccaacgtaagcgatagcagagatagccacgatatctctcaccacgtaagacatagacttcacgagagatctctcgtaacagtgcttagggatagcgtcaaggatatccttgatggtgtaatctggcaccttgaaaacgtttccgaaggtatcgatagcggtcttttgctgcttgaaagatgcaacgtttccagaacgcctaacggtcttagtagatccctcaaggatctcagatccagacacggtaaccttagacatggtatggtaattgtaaatgtaattgtaatgttgtttgttgtttgttgttgttggtaattgttgtaaaatttttggtggtgattggttctttaaggtgtgagagtgagttgtgagttgtgtggtgggtttggtgagattggggatggtgggtttatatagtggagactgaggaatggggtcgtgagtgttaactttgcatgggctacacgtgggttcttttgggcttacacgtagtattattcatgcaaatgcagccaatacatatacggtattttaataatgtgtgggaatacaatatgccgagtattttactaattttggcaatgacaagtgtacatttggattatcttacttggcctctcttgctttaatttggattatttttattctcttaccttggccgttcatattcacatccctaaaggcaagacagaattgaatggtggccaaaaattaaaacgatggatatgacctacatagtgtaggatcaattaacgtcgaaggaaaatactgattctgcccgttcgactcagatcttccaaggcctcgtctccgagtccgctgcttctcgccgcgccgatcacttctccgccgccaacaaggcttgtagttaataggaatcattcagggattgtgattccgggcagtagtaattaataatatagtattagtatacagaacctcttatttagctaaaagattatgttcttaatgttgataagaagtttgagaaacaaatataattgagcttctgattagttgatcgtaattggtcattaataattgtatctaaccagtgcagtataagagcgtataagagcatcttcaaaaagactttattttagagttaatcagtgcagtataagagcatctctaaaaaaactctaattatagagttttgcaaactctatatttgaagttttaaggtgtttttttttcaaaagcaaaacttcaaatttaacttcaaaattatttgtaatttacactatgctctttatatttatcataattaatataagggggtgttagtgggacttagatttctatagagtttgttgattttaaaagttgagagatttgttaaatttagaaagagatgtagagaattttgtctattgtgaaaatctatgaaaatagagtaatgtaatgattctaagaattcaaagtaaacatgtagtattctcaaaatctaaatttgtgaaacagtggtcccagattttcaagactcagactaaaggctatggaggaagctagggttttggcgattggcgacactagggtttcgagtacggcagatttggatgaaactatgatggatgtgggggagagagggagaccgccaggagatccgccagataagttaacctcatgggtagcgaaggtggtggagacggctgagggagggatgccagtaccggaggttttgattgcagattcttttgtgtcggagagggtacgggtagaatttccgaatg

SEQ ID NO: 41 - DNA, 49789 bp, synthetic construct
  misc_feature 1..49789: note = Chimeric 16 transgene inserted into Brassica
  source 1..49789: mol_type = other DNA
aaaaaatacaaccaaagaaaaatataccagaaggttgtgatttggtccattatataaaaattacgaaatgaatttctttatccttttatctcaaattttattgaagacttttgtaggattatagttgactttatgctcacatatatatacactgatcaaaactttttaaaaacataaagaaattgtgaaacaataaaaataaaatgaaatgagtaattaatgagtagattaagacattggaccctccacaggcgataaagtaaaataatcagaagttgcaggaggcaaaggaggactactactaatacttggaacttggaagtagctatcgtgcgcatctgcctccaagtccaacaccttataacaaatttccgccgggaagaaagaaaagtctctctgccctctcttctttagcctccagcttctgcaaaccatacgtacaaacaagatagacacaatcctccctacctccttcttctatcttcatcgaaagattcaaccaccactcaagtcttctctctcttttttggaaagaaaaaaggtaaaagctttcttctttctgagcaaactcccatgaatttcccttttgggggtttagggtctttccttttatgttcctacttcggtataattcgatttcatgcgaacttagattataaaaatttgatcttttttttgtggggtttgaaattgaaatccattttaggggttaccatcgttgaccaaatgtctcgactttgttcgaatcatgatgttacttaatcatggaggagaagaaggatttttataaccatgtctctgttgcttgctgcttaaaccctatataattggaaactttttgttttagtctgtgtctgaaagtttctatattcgtattgtctattttgtaaagactaaaacaaaaatgcctatttttagtttgttcttgttccgcaacaccgttactgaactcttcgttcacttaaacagtttgtgtgtgtgagaaacagcgtaatgagctgctttggttgttgtggtggtgacgattttcgtcgagttgctgaaactggacccaagccagtgtacggcgcaggaggtactttaagcttataaccctttgtctatcctttggctagcggctaatgttgatgaacttttttattcaaccgttggctaaggtaacactgatagtttaaactgaaggcgggaaacgacaatctgctagtggatctcccagtcacgacgttgtaaaacgggcgccccgcggaaagcttgcggccgcggtaccgcccgttcgactcagatcttccaaggcctcgtctccgagtccgctgcttctcgccgcgccgatcacttctccgccgccaacaaggcttgtagttaataggaatcattcagggattgtgattccgggcagtagtaattaataatatagtattagtatagataatatgtttcgtttgggatctttggaacgttgctctgttccttgttgttcattttaaagcttttgagggatagttgcagaactgttcggtgatgcttcatcctctcaagaactagatttgggtaaagaaacatccatgcatggatatggaatgttgttcttccgattggagattattttataaaatttaaaattcatgatttaaaaaaacacataaaaaccacaaaattcatgatttattgacaatacgatacaaaattagcaccaccggctactggctcattacacatttccccttcccctcattctcactttgtggctttattattattattattacatatattttaccgttattatttcacgtcacataagcttgttaattaatcattagtgagccttctcagcctttccgttaacgtagtagtgctgtcccaccttatcaaggttagagaaagtagccttccaagcaccgtagtaagagagcaccttgtagttgagtccccacttcttagcgaaaggaacgaatcttctgctaacctcaggctgtctgaattgaggcatatcagggaagaggtggtggataacctgacagttaaggtatcccataagccagttcacgtatcctctagaaggatcgatatcaacggtgtgatcaacagcgtagttaacccaagaaaggtgcttatcagatggaacaacagggaggtgagtatgagaagtagagaagtgagcgaaaaggtacatgtaagcgatccagtttccgaaagtgaaccaccagtaagcaacaggccaagagtatccagtagcaagcttgataacagcggttctaacaacatgagaaacgagcatccaagaagcctcttcgtagttcttcttacggagaacttgtctagggtggagaacgtagatccagaaagcttgaacaagaagtccagaggtaacaggaacgaaagtccaagcttgaagtctagcccaagctctagagaatcctctaggtctgttatcctcaacagcagtgttgaagaaagccacagcaggagtggtatcaagatccatatcgtgtctaaccttttgaggggtagcatggtgcttgttatgcatctggttccacatctcaccagaagtagaaagtccgaatccacaagtcatagcctgaagtctcttgtccacgtaaacagatccggtaagagagttatgtccaccctcatgttgaacccatccacatctagctccgaagaaagcaccgtaaacaacagaagcaatgatagggtatccagcgtacataagagcagttccaagagcgaatgtagcaagaagctcgagaagtctgtaagccacatgggtgatagaaggcttgaagaatccatctctctcaagctcagcacgccatctagcgaaatcctcaagcataggagcatcctcagactcagatctcttgatctcagcaggtctagaaggcaaagctctaagcatcttccaagccttgagagaacgcatgtggaattctttgaaagcctcagtagcatcagcaccagtgttagcaagcatgtagaagatcacagatccaccagggtgcttgaagttagtcacatcgtactcaacgtcctcaactctaacccatctagtctcgaaagtagcagcaagctcatgaggctcaagagtcttaagatcaacaggagcagtagaagcatccttagcatcaagagcctcagcagaagatttagacctggtaagtggagatctaggagaagatcttccatcagtcttaggagggcacatggtatggtaattgtaaatgtaattgtaatgttgtttgttgtttgttgttgttggtaattgttgtaaaattaattaagtgggtatcttttggatggataagcaagtagtgatgatgttctaggtgaagtgatgggggtgttttatagcgggagatggtgaaatggatggtcgccacataagaaatggaggggaagggttcttgcgccattcttcagtttgcatggatgcatgggtttcattttgtaacacgtaataaggacaatgaagtgcaggtgtctctcaagtttcagaggggatatgtggacagaagaagaacggcgatgatattgatggaaatggccatctagtgtgaatctattcggttgataatactagtgcattttggccgttaatcccttcaattaactgcacaaacttcagttgagtattgattatttgattataggttctgtaaacacaataccaagtttatttagaggggagacatacaaatagtttcgatataaataatagagtggttaaacttagttattaaaactatatataaagtctaaaagttaaattatttttttaattgcaaatatataaagtctaaaggggttacattatttcttaagagatgtaactctgttggaatctgacttaatccgtctcatcactctggtttccagttctaatctaatgaattgttttctgccaaagaatttgaagcaagaagtaaattgatcaatgccgtcaacccacaccaaaccgtcaacccactaccatcgccgcggagacccccaaactcaacctccacccatcggtaagaagcacagggcagcccgcaccaccaccaatttggcgtgcatgacacctagggacttggcacgggaggcggcgcacgtggatgcaaatgacgggatatcagatgacaggaaacgacgttgagagaccatacgatgtagaatatgagctcaccatcaacgagaaactaggaaaatcacaaaaaaaacaactctcgtaattgtacgagtggcacagatgggtctgcctcaacatatctctaatacggcgaagcctgcccaacacgtagttgccggaatccggtgtggagctcacgactctgaaagataggcgcttcctgtttcgtttcgctcacccactggacgtccgtcatgtgatggatttcggtcattggtttgctgacaaccacattctgaagctccatgagatgagtcttcacaataggtcctgctcaataccgtggagttatggttgcaagtccataacttgccgttcgaatattttgcggagccagtcggacgggaattggcgagctcggctgacacctataaaggccatgacaagaagaaccaaaagttcttccctaatgctttcatgaggcttcgggtcgttatggatgtcggaaaacccctcttgaaggaacgagacgttattatgcatgacggtaagactattacttgtcagtataagtatgaaagattacctgtcttctgctttgtttgtggattgattggacacgttgaaaaaaaatgtgcacttcgatttcaatactcagagatcgacttcccttttctctaggagtattcgatcaaggcattaacatggaaggaagctcaagctctaaaggcttcacaatggaacctgaaaaatttcaacaagcctaaactgaaatcgaagtcaaatcacccaaccgggagctctaaatcagcaaacactcctcctccacagtatccaatcatcgtgcacgatgctccaggtattgcaagccaggtattgcaagctaggagtaggatagagaccttaaacgtcgttggtgtgaagagtcatcttcagacctaatggagatagatgtagacggcggcacgaagactctgaaacaccagaaaggctagtccaggataaggatctgctatcccaactgacctctcgttagtcccaaggcctctcaactagagcaggaggaaggatggtcacaagactaggataatgatgtttccaatatgaacctgaatgtccatagctaatttttttagtcttgcttctgcactttttgtttattatgttctggtgactatgttatttacccttgtccgtatgcttgagggtaccctagtagattggttggttggtttccatgtaccagaaggcttaccctattagttgaaagttgaaactttgttccctactcaattcctagttgtgtaaatgtatgtatatgtaatgtgtataaaacgtagtacttaaatgactaggagtggttcttgagaccgatgagagatgggagcagaactaaagatgatgacataattaagaacgaatttgaaaggctcttaggtttgaatcctattcgagaatgtttttgtcaaagatagtggcgattttgaaccaaagaaaacatttaaaaaatcagtatccggttacgttcatgcaaatagaaagtggtctaggatctgattgtaattttagacttaaagagtctcttaagattcaatcctggctgtgtacaaaactacaaataatatattttagactatttggccttaactaaacttccactcattatttactgaggttagagaatagacttgcgaataaacacattcccgagaaatactcatgatcccataattagtcagagggtatgccaatcagatctaagaacacacattccctcaaattttaatgcacatgtaatcatagtttagcacaattcaaaaataatgtagtattaaagacagaaatttgtagacttttttttggcgttaaaagaagactaagtttatacgtacattttattttaagtggaaaaccgaaattttccatcgaaatatatgaatttagtatatatatttctgcaatgtactattttgctattttggcaactttcagtggactactactttattacaatgtgtatggatgcatgagtttgagtatacacatgtctaaatgcatgctttgtaaaacgtaacggaccacaaaagaggatccatacaaatacatctcatagcttcctccattattttccgacacaaacagagcattttacaacaattaccaacaacaacaaacaacaaacaacattacaattacatttacaattaccataccatggcctctatcgctatccctgctgctcttgctggaactcttggatacgttacctacaatgtggctaaccctgatatcccagcttctgagaaagttcctgcttacttcatgcaggttgagtactggggacctactatcggaactattggatacctcctcttcatctacttcggaaagcgtatcatgcagaacagatctcaacctttcggactcaagaacgctatgctcgtttacaacttctaccagaccttcttcaacagctactgcatctaccttttcgttacttctcatagggctcagggacttaaggtttggggaaacatccctgatatgactgctaactcttggggaatctctcaggttatctggcttcactacaacaacaagtacgttgagcttctcgacaccttcttcatggtgatgaggaagaagttcgaccagctttctttccttcacatctaccaccacactcttctcatctggtcatggttcgttgttatgaagcttgagcctgttggagattgctacttcggatcttctgttaacaccttcgtgcacgtgatcatgtactcttactacggacttgctgctcttggagttaactgtttctggaagaagtacatcacccagatccagatgcttcagttctgtatctgtgcttctcactctatctacaccgcttacgttcagaataccgctttctggcttccttaccttcaactctgggttatggtgaacatgttcgttctcttcgccaacttctaccgtaagaggtacaagtctaagggtgctaagaagcagtgataaggcgcgcggcgcgccgggccgccgccatgtgacagatcgaaggaagaaagtgtaataagacgactctcactactcgatcgctagtgattgtcattgttatatataataatgttatctttcacaacttatcgtaatgcatgtgaaactataacacattaatcctacttgtcatatgataacactctccccatttaaaactcttgtcaatttaaagatataagattctttaaatgattaaaaaaaatatattataaattcaatcactcctactaataaattattaattattatttattgattaaaaaaatacttatactaatttagtctgaatagaataattagattctagtctcatccccttttaaaccaacttagtaaacgtttttttttttaattttatgaagttaagtttttaccttgtttttaaaaagaatcgttcataagatgccatgccagaacattagctacacgttacacatagcatgcagccgcggagaattgtttttcttcgccacttgtcactcccttcaaacacctaagagcttctctctcacagcacacacatacaatcacatgcgtgcatgcattattacacgtgatcgccatgcaaatctcctttatagcctataaattaactcatccgcttcactctttactcaaaccaaaactcatcgatacaaacaagattaaaaacatacacgaggatcttttacaacaattaccaacaacaacaaacaacaaacaacattacaattacatttacaattaccataccatgcctccaagggactcttactcttatgctgctcctccttctgctcaacttcacgaagttgatactcctcaagagcacgacaagaaagagcttgttatcggagatagggcttacgatgttaccaacttcgttaagagacaccctggtggaaagatcattgcttaccaagttggaactgatgctaccgatgcttacaagcagttccatgttagatctgctaaggctgacaagatgcttaagtctcttccttctcgtcctgttcacaagggatactctccaagaagggctgatcttatcgctgatttccaagagttcaccaagcaacttgaggctgagggaatgttcgagccttctcttcctcatgttgcttacagacttgctgaggttatcgctatgcatgttgctggtgctgctcttatctggcatggatacactttcgctggaatcgctatgcttggagttgttcagggaagatgtggatggcttatgcatgagggtggacattactctctcactggaaacattgctttcgacagagctatccaagttgcttgttacggacttggatgtggaatgtctggtgcttggtggcgtaaccagcataacaagcaccatgctactcctcaaaagcttcagcacgatgttgatcttgatacccttcctctcgttgctttccatgagagaatcgctgctaaggttaagtctcctgctatgaaggcttggctttctatgcaagctaagcttttcgctcctgttaccactcttcttgttgctcttggatggcagctttaccttcatcctagacacatgctcaggactaagcactacgatgagcttgctatgctcggaatcagatacggacttgttggataccttgctgctaactacggtgctggatacgttctcgcttgttaccttctttacgttcagcttggagctatgtacatcttctgcaacttcgctgtttctcatactcacctccctgttgttgagcctaacgagcatgctacttgggttgagtacgctgctaaccacactactaactgttctccatcttggtggtgtgattggtggatgtcttaccttaactaccagatcgagcaccacctttacccttctatgcctcaattcagacaccctaagatcgctcctagagttaagcagcttttcgagaagcacggacttcactacgatgttagaggatacttcgaggctatggctgatactttcgctaaccttgataacgttgcccatgctcctgagaagaaaatgcagtaatgagatcgttcaaacatttggcaataaagtttcttaagattgaatcctgttgccggtcttgcgatgattatcatataatttctgttgaattacgttaagcacgtaataattaacatgtaatgcatgacgttatttatgagatgggtttttatgattagagtcccgcaattatacatttaatacgcgatagaaaacaaaatatagcgcgcaaactaggataaattatcgcgcgcggtgtcatctatgttactagatcggtcgattaaaaatcccaattatatttggtctaatttagtttggtattgagtaaaacaaattcgaaccaaaccaaaatataaatatatagtttttatatatatgcctttaagactttttatagaattttctttaaaaaatatctagaaatatttgcgactcttctggcatgtaatatttcgttaaatatgaagtgctccatttttattaactttaaataattggttgtacgatcactttcttatcaagtgttactaaaatgcgtcaatctctttgttcttccatattcatatgtcaaaatctatcaaaattcttatatatctttttcgaatttgaagtgaaatttcgataatttaaaattaaatagaacatatcattatttaggtatcatattgatttttatacttaattactaaatttggttaactttgaaagtgtacatcaacgaaaaattagtcaaacgactaaaataaataaatatcatgtgttattaagaaaattctcctataagaatattttaatagatcatatgtttgtaaaaaaaattaatttttactaacacatatatttacttatcaaaaatttgacaaagtaagattaaaataatattcatctaacaaaaaaaaaaccagaaaatgctgaaaacccggcaaaaccgaaccaatccaaaccgatatagttggtttggtttgattttgatataaaccgaaccaactcggtccatttgcacccctaatcataatagctttaatatttcaagatattattaagttaacgttgtcaatatcctggaaattttgcaaaatgaatcaagcctatatggctgtaatatgaatttaaaagcagctcgatgtggtggtaatatgtaatttacttgattctaaaaaaatatcccaagtattaataatttctgctaggaagaaggttagctacgatttacagcaaagccagaatacaaagaaccataaagtgattgaagctcgaaatatacgaaggaacaaatatttttaaaaaaatacgcaatgacttggaacaaaagaaagtgatatattttttgttcttaaacaagcatcccctctaaagaatggcagttttcctttgcatgtaactattatgctcccttcgttacaaaaattttggactactattgggaacttcttctgaaaatagtgatagaacccacacgagcatgtgctttccatttaattttaaaaaccaagaaacatacatacataacattccatcagcctctctctctttttattacggttaatgacttaaaacacatcttattatcccatccttaacacctagcagtgtctttatacgatctcatcgatcaccacttcaaaaccatgcagactgctgctgcccctggagctggcatcggctaggctgggtgccgcactgtcccggaaggtccctagcgacttgtttagattgatgggaccacctctcaacttcctgctgctgtccctgctgctggatgtcctgcctcatctggccgattgcacgctccagtcccctgcatgtgcactcgctcctcaattgcttaagatcatcgcagcagctatcgaagtgctggctctgttgccctcctccacggccttggttgtagtagtagctgccgccgcccttctggactttttcccacaggaaccgccgaataattcgatagaaccacacgagcatgtgctttcatttattttaaaaaccaagaaacatacataacatttcatcagcctctctctctctctctctctctctctctctctctctctctctctctctctctttattacagctgttacactaacttaaaacacattcatctcattattattattattatccatccttaacacctagcagtgtctttgtacgatctcataatcgatcaccccttcatcaggtatccttaggcttcactccaacgttgttgcagttacggaacatgtacacaccatcatggttctcaacgaactggcaagatctccaagttttccaaaggctaacccacatgttctcatcggtgtgtctgtagtgctctcccataactttcttgatgcactcggtagcttctctagcatggtagaatgggatccttgaaacgtagtgatggagcacatgagtctcgatgatgtcatggaagatgattccgaggattccgaactctctatcgatagtagcagcagcacccttagcgaaagtccactcttgagcatcgtaatgaggcatagaagaatcggtgtgctgaaggaaggtaacgaaaacaagccagtggttaacaaggatccaaggacagaaccatgtgatgaaagtaggccagaatccgaaaaccttgtaagcggtgtaaacagaagtgagggtagcaaggattccaagatcagaaagaacgatgtaccagtagtccttcttatcgaaaacagggctagaaggccagtagtgagacttgaagaacttagaaacaccagggtaaggttgtccagtagcgttagtagcaaggtaaagagaaagtcctccaagctgttggaacaagagagcgaaaacagagtagataggagtttcctcagcgatatcgtgaaggctggtaacttggtgcttctctttgaattcctcggcggtgtaaggaacgaaaaccatatctctggtcatgtgtccagtagccttatggtgcttagcatgagagaacttccagctgaagtaaggaaccataacaagagagtggagaacccatccaacggtatcgttaacccatccgtagttagagaaagcagaatgtccacactcatgtccaaggatccagattccgaatccgaaacaagagatagagaacacgtaagcagaccaagcagcgaatctaaggaattcgttagggagaagagggatgtaggtaagtccaacgtaagcgatagcagagatagccacgatatctctcaccacgtaagacatagacttcacgagagatctctcgtaacagtgcttagggatagcgtcaaggatatccttgatggtgtaatctggcaccttgaaaacgtttccgaaggtatcgatagcggtcttttgctgcttgaaagatgcaacgtttccagaacgcctaacggtcttagtagatccctcaaggatctcagatccagacacggtaaccttagacatggtatggtaattgtaaatgtaattgtaatgttgtttgttgtttgttgttgttggtaattgttgtaaaatttttggtggtgattggttctttaaggtgtgagagtgagttgtgagttgtgtggtgggtttggtgagattggggatggtgggtttatatagtggagactgaggaatggggtcgtgagtgttaactttgcatgggctacacgtgggttcttttgggcttacacgtagtattattcatgcaaatgcagccaatacatatacggtattttaataatgtgtgggaatacaatatgccgagtattttactaattttggcaatgacaagtgtacatttggattatcttacttggcctctcttgctttaatttggattatttttattctcttaccttggccgttcatattcacatccctaaaggcaagacagaattgaatggtggccaaaaattaaaacgatggatatgacctacatagtgtaggatcaattaacgtcgaaggaaaatactgattctctcaagcatacggacaagggtaaataacatagtcaccagaacataataaacaaaaagtgcagaagcaagactaaaaaaattagctatggacattcaggttcatattggaaacatcattatcctagtcttgtgaccatccttcctcctgctctagttgagaggccttgggactaacgagaggtcagttgggatagcagatccttatcctggactagcctttctggtgtttcagagtcttcgtgccgccgtctacatctatctccattaggtctgaagatgactcttcacaccaacgacgtttaaggtctctatcctactcctagcttgcaatacctggcttgcaatacctggagcatcgtgcacgatgattggatactgtggaggaggagtgtttgctgatttagagctcccggttgggtgatttgacttcgatttcagtttaggcttgttgaaatttttcaggttccattgtgaagcctttagagcttgagcttccttccatgttaatgccttgatcgaatactcctagagaaaagggaagtcgatctctgagtattgaaatcgaagtgcacattttttttcaacgtgtccaatcaatccacaaacaaagcagaagacaggtaatctttcatacttatactgacaagtaatagtcttaccgtcatgcataataacgtctcgttccttcaagaggggttttccgacatccataacgacccgaagcctcatgaaagcattagggaagaacttttggttcttcttgtcatggcctttataggtgtcagccgagctcgccaattcccgtccgactggctccgcaaaatattcgaacggcaagttatggacttgcaaccataactccacggtattgagcaggacctattgtgaagactcatctcatggagcttcagaatgtggttgtcagcaaaccaatgaccgaaatccatcacatgacggacgtccagtgggtgagcgaaacgaaacaggaagcgcctatctttcagagtcgtgagctccacaccggattccggcaactacgtgttgggcaggcttcgccgtattagagatatgttgaggcagacccatctgtgccactcgtacaattacgagagttgttttttttgtgattttcctagtttctcgttgatggtgagctcatattctacatcgtatggtctctcaacgtcgtttcctgtcatctgatatcccgtcatttgcatccacgtgcgccgcctcccgtgccaagtccctaggtgtcatgcacgccaaattggtggtggtgcgggctgccctgtgcttcttaccgatgggtggaggttgagtttgggggtctccgcggcgatggtagtgggttgacggtttggtgtgggttgacggcattgatcaatttacttcttgcttcaaattctttggcagaaaacaattcattagattagaactggaaaccagagtgatgagacggattaagtcagattccaacagagttacatctcttaagaaataatgtaacccctttagactttatatatttgcaattaaaaaaataatttaacttttagactttatatatagttttaataactaagtttaaccactctattatttatatcgaaactatttgtatgtctcccctctaaataaacttggtattgtgtttacagaacctataatcaaataatcaatactcaactgaagtttgtgcagttaattgaagggattaacggccaaaatgcactagtattatcaaccgaatagattcacactagatggccatttccatcaatatcatcgccgttcttcttctgtccacatatcccctctgaaacttgagagacacctgcacttcattgtccttattacgtgttacaaaatgaaacccatgcatccatgcaaactgaagaatggcgcaagaacccttcccctccatttcttatgtggcgaccatccatttcaccatctcccgctataaaacacccccatcacttcacctagaacatcatcactacttgcttatccatccaaaagatacccacttttacaacaattaccaacaacaacaaacaacaaacaacattacaattacatttacaattaccataccatgccacctagcgctgctaagcaaatgggagcttctactggtgttcatgctggtgttactgactcttctgctttcaccagaaaggatgttgctgatagacctgatctcaccatcgttggagattctgtttacgatgctaaggctttcagatctgagcatcctggtggtgctcatttcgtttctttgttcggaggaagagatgctactgaggctttcatggaataccatagaagggcttggcctaagtctagaatgtctagattccacgttggatctcttgcttctactgaggaacctgttgctgctgatgagggataccttcaactttgtgctaggatcgctaagatggtgccttctgtttcttctggattcgctcctgcttcttactgggttaaggctggacttatccttggatctgctatcgctcttgaggcttacatgctttacgctggaaagagacttctcccttctatcgttcttggatggcttttcgctcttatcggtcttaacatccagcatgatgctaaccatggtgctttgtctaagtctgcttctgttaaccttgctcttggactttgtcaggattggatcggaggatctatgatcctttggcttcaagagcatgttgttatgcaccacctccacactaacgatgttgataaggatcctgatcaaaaggctcacggtgctcttagactcaagcctactgatgcttggtcacctatgcattggcttcagcatctttaccttttgcctggtgagactatgtacgctttcaagcttttgttcctcgacatctctgagcttgttatgtggcgttgggagggtgagcctatctctaagcttgctggatacctctttatgccttctttgcttctcaagcttaccttctgggctagattcgttgctttgcctctttaccttgctccttctgttcatactgctgtgtgtatcgctgctactgttatgactggatctttctacctcgctttcttcttcttcatctcccacaacttcgagggtgttgcttctgttggacctgatggatctatcacttctatgactagaggtgctagcttccttaagagacaagctgagacttcttctaacgttggaggacctcttcttgctactcttaacggtggactcaactaccaaattgagcatcacttgttccctagagttcaccatggattctaccctagacttgctcctcttgttaaggctgagcttgaggctagaggaatcgagtacaagcactaccctactatctggtctaaccttgcttctaccctcagacatatgtacgctcttggaagaaggcctagatctaaggctgagtaatgacaagcttatgtgacgtgaaataataacggtaaaatatatgtaataataataataataaagccacaaagtgagaatgaggggaaggggaaatgtgtaatgagccagtagccggtggtgctaattttgtatcgtattgtcaataaatcatgaattttgtggtttttatgtgtttttttaaatcatgaattttaaattttataaaataatctccaatcggaagaacaacattccatatccatgcatggatgtttctttacccaaatctagttcttgagaggatgaagcatcaccgaacagttctgcaactatccctcaaaagctttaaaatgaacaacaaggaacagagcaacgttccaaagatcccaaacgaaacatattatctatactaatactatattattaattactactgcccggaatcacaatccctgaatgattcctattaactacaagccttgttggcggcggagaagtgatcggcgcggcgagaagcagcggactcggagacgaggccttggaagatctgagtcgaacgggcagaatcagtattttccttcgacgttaattgatcctacactatgtaggtcatatccatcgttttaatttttggccaccattcaattctgtcttgcctttagggatgtgaatatgaacggccaaggtaagagaataaaaataatccaaattaaagcaagagaggccaagtaagataatccaaatgtacacttgtcattgccaaaattagtaaaatactcggcatattgtattcccacacattattaaaataccgtatatgtattggctgcatttgcatgaataatactacgtgtaagcccaaaagaacccacgtgtagcccatgcaaagttaacactcacgaccccattcctcagtctccactatataaacccaccatccccaatctcaccaaacccaccacacaactcacaactcactctcacaccttaaagaaccaatcaccaccaaaaattttacaacaattaccaacaacaacaaacaacaaacaacattacaattacatttacaattaccataccatgagcgctgttaccgttactggatctgatcctaagaacagaggatcttctagcaacaccgagcaagaggttccaaaagttgctatcgataccaacggaaacgtgttctctgttcctgatttcaccatcaaggacatccttggagctatccctcatgagtgttacgagagaagattggctacctctctctactacgtgttcagagatatcttctgcatgcttaccaccggataccttacccataagatcctttaccctctcctcatctcttacacctctaacagcatcatcaagttcactttctgggccctttacacttacgttcaaggacttttcggaaccggaatctgggttctcgctcatgagtgtggacatcaagctttctctgattacggaatcgtgaacgatttcgttggatggacccttcactcttaccttatggttccttacttcagctggaagtactctcatggaaagcaccataaggctactggacacatgaccagagatatggttttcgttcctgccaccaaagaggaattcaagaagtctaggaacttcttcggtaacctcgctgagtactctgaggattctccacttagaaccctttacgagcttcttgttcaacaacttggaggatggatcgcttacctcttcgttaacgttacaggacaaccttaccctgatgttccttcttggaaatggaaccacttctggcttacctctccacttttcgagcaaagagatgctctctacatcttcctttctgatcttggaatcctcacccagggaatcgttcttactctttggtacaagaaattcggaggatggtcccttttcatcaactggttcgttccttacatctgggttaaccactggctcgttttcatcacattccttcagcacactgatcctactatgcctcattacaacgctgaggaatggactttcgctaagggtgctgctgctactatcgatagaaagttcggattcatcggacctcacatcttccatgatatcatcgagactcatgtgcttcaccactactgttctaggatcccattctacaacgctagacctgcttctgaggctatcaagaaagttatgggaaagcactacaggtctagcgacgagaacatgtggaagtcactttggaagtctttcaggtcttgccaatacgttgacggtgataacggtgttctcatgttccgtaacatcaacaactgcggagttggagctgctgagaagtaatgaaggggtgatcgattatgagatcgtacaaagacactgctaggtgttaaggatggataataataataataatgagatgaatgtgttttaagttagtgtaacagctgtaataaagagagagagagagagagagagagagagagagagagagagagagagagagaggctgatgaaatgttatgtatgtttcttggtttttaaaataaatgaaagcacatgctcgtgtggttctatcgaattattcggcggttcctgtgggaaaaagtccagaagggccgccgcagctactactacaaccaaggccgtggaggagggcaacagagccagcacttcgatagctgctgcgatgatcttaagcaattgaggagcgagtgcacatgcaggggactggagcgtgcaatcggccagatgaggcaggacatccagcagcagggacagcagcaggaagttgagaggtggtcccatcaatctaaacaagtcgctagggaccttccgggacagtgcggcacccagcctagccgatgccagctccaggggcagcagcagtctgcatggttttgaagtggtgatcgatgagatcgtataaagacactgctaggtgttaaggatgggataataagatgtgttttaagtcattaaccgtaataaaaagagagagaggctgatggaatgttatgtatgtatgtttcttggtttttaaaattaaatggaaagcacatgctcgtgtgggttctatctcgattaaaaatcccaattatatttggtctaatttagtttggtattgagtaaaacaaattcgaaccaaaccaaaatataaatatatagtttttatatatatgcctttaagactttttatagaattttctttaaaaaatatctagaaatatttgcgactcttctggcatgtaatatttcgttaaatatgaagtgctccatttttattaactttaaataattggttgtacgatcactttcttatcaagtgttactaaaatgcgtcaatctctttgttcttccatattcatatgtcaaaatctatcaaaattcttatatatctttttcgaatttgaagtgaaatttcgataatttaaaattaaatagaacatatcattatttaggtatcatattgatttttatacttaattactaaatttggttaactttgaaagtgtacatcaacgaaaaattagtcaaacgactaaaataaataaatatcatgtgttattaagaaaattctcctataagaatattttaatagatcatatgtttgtaaaaaaaattaatttttactaacacatatatttacttatcaaaaatttgacaaagtaagattaaaataatattcatctaacaaaaaaaaaaccagaaaatgctgaaaacccggcaaaaccgaaccaatccaaaccgatatagttggtttggtttgattttgatataaaccgaaccaactcggtccatttgcacccctaatcataatagctttaatatttcaagatattattaagttaacgttgtcaatatcctggaaattttgcaaaatgaatcaagcctatatggctgtaatatgaatttaaaagcagctcgatgtggtggtaatatgtaatttacttgattctaaaaaaatatcccaagtattaataatttctgctaggaagaaggttagctacgatttacagcaaagccagaatacaaagaaccataaagtgattgaagctcgaaatatacgaaggaacaaatatttttaaaaaaatacgcaatgacttggaacaaaagaaagtgatatattttttgttcttaaacaagcatcccctctaaagaatggcagttttcctttgcatgtaactattatgctcccttcgttacaaaaattttggactactattgggaacttcttctgaaaatagtcctgcaggctagtagattggttggttggtttccatgtaccagaaggcttaccctattagttgaaagttgaaactttgttccctactcaattcctagttgtgtaaatgtatgtatatgtaatgtgtataaaacgtagtacttaaatgactaggagtggttcttgagaccgatgagagatgggagcagaactaaagatgatgacataattaagaacgaatttgaaaggctcttaggtttgaatcctattcgagaatgtttttgtcaaagatagtggcgattttgaaccaaagaaaacatttaaaaaatcagtatccggttacgttcatgcaaatagaaagtggtctaggatctgattgtaattttagacttaaagagtctcttaagattcaatcctggctgtgtacaaaactacaaataatatattttagactatttggccttaactaaacttccactcattatttactgaggttagagaatagacttgcgaataaacacattcccgagaaatactcatgatcccataattagtcagagggtatgccaatcagatctaagaacacacattccctcaaattttaatgcacatgtaatcatagtttagcacaattcaaaaataatgtagtattaaagacagaaatttgtagacttttttttggcgttaaaagaagactaagtttatacgtacattttattttaagtggaaaaccgaaattttccatcgaaatatatgaatttagtatatatatttctgcaatgtactattttgctattttggcaactttcagtggactactactttattacaatgtgtatggatgcatgagtttgagtatacacatgtctaaatgcatgctttgtaaaacgtaacggaccacaaaagaggatccatacaaatacatctcatagcttcctccattattttccgacacaaacagagcattttacaacaattaccaacaacaacaaacaacaaacaacattacaattacatttacaattaccataccatggaatttgctcaacctctcgttgctatggctcaagagcagtacgctgctatcgatgctgttgttgctcctgctatcttctctgctaccgactctattggatggggactcaagcctatctcttctgctactaaggatctccctctcgttgaatctcctacccctcttatcctttctctcctcgcttacttcgctatcgttggttctggactcgtttaccgtaaagtgttccctagaaccgttaagggacaggatcctttccttctcaaggctcttatgctcgctcacaacgttttccttatcggactcagcctttacatgtgcctcaagctcgtttacgaggcttacgtgaacaagtactccttctggggaaacgcttacaaccctgctcaaaccgagatggctaaggtgatctggatcttctacgtgtccaagatctacgagttcatggacaccttcatcatgcttctcaagggaaacgttaaccaggtttccttcctccatgtttaccaccacggatctatctctggaatctggtggatgatcacttatgctgctccaggtggagatgcttacttctctgctgctctcaactcttgggttcatgtgtgcatgtacacctactacttcatggctgctgttcttcctaaggacgaaaagaccaagagaaagtacctttggtggggaagataccttacccagatgcaaatgttccagttcttcatgaaccttctccaggctgtttacctcctctactcttcttctccttaccctaagttcattgctcaactcctcgttgtttacatggttaccctcctcatgcttttcggaaacttctactacatgaagcaccacgcttctaagtgataagggccgccgccatgtgacagatcgaaggaagaaagtgtaataagacgactctcactactcgatcgctagtgattgtcattgttatatataataatgttatctttcacaacttatcgtaatgcatgtgaaactataacacattaatcctacttgtcatatgataacactctccccatttaaaactcttgtcaatttaaagatataagattctttaaatgattaaaaaaaatatattataaattcaatcactcctactaataaattattaattattatttattgattaaaaaaatacttatactaatttagtctgaatagaataattagattctagcctgcagggcggccgcggatcccatggagtcaaagattcaaatagaggacctaacagaactcgccgtaaagactggcgaacagttcatacagagtctcttacgactcaatgacaagaagaaaatcttcgtcaacatggtggagcacgacacacttgtctactccaaaaatatcaaagatacagtctcagaagaccaaagggcaattgagacttttcaacaaagggtaatatccggaaacctcctcggattccattgcccagctatctgtcactttattgtgaagatagtggaaaaggaaggtggctcctacaaatgccatcattgcgataaaggaaaggccatcgttgaagatgcctctgccgacagtggtcccaaagatggacccccacccacgaggagcatcgtggaaaaagaagacgttccaaccacgtcttcaaagcaagtggattgatgtgatatctccactgacgtaagggatgacgcacaatcccactatccttcgcaagacccttcctctatataaggaagttcatttcatttggagagaacacgggggactgaattaaatatgagccctgagaggcgtcctgttgaaatcagacctgctactgctgctgatatggctgctgtttgtgatatcgtgaaccactacatcgagacttctaccgttaacttcagaactgagcctcaaactcctcaagagtggatcgatgatcttgagagactccaagatagatacccttggcttgttgctgaggttgagggtgttgttgctggaatcgcttacgctggaccttggaaggctagaaacgcttacgattggactgttgagtctaccgtttacgtttcacacagacatcagagacttggacttggatctaccctttacactcaccttctcaagtctatggaagctcagggattcaagtctgttgttgctgttatcggactccctaacgatccttctgttagacttcatgaggctcttggatacactgctagaggaactcttagagctgctggatacaagcacggtggatggcatgatgttggattctggcaaagagatttcgagcttcctgctcctcctagacctgttagaccagttactcagatctgaatttgcgtgatcgttcaaacatttggcaataaagtttcttaagattgaatcctgttgccggtcttgcgatgattatcatataatttctgttgaattacgttaagcatgtaataattaacatgtaatgcatgacgttatttatgagatgggtttttatgattagagtcccgcaattatacatttaatacgcgatagaaaacaaaatatagcgcgcaaactaggataaattatcgcgcgcggtgtcatctatgttactagatcactagtgatgtacggttaaaaccaccccagtacattaaaaacgtccgcaatgtgttattaagttgtctaagcgtcaatttgtttacaccacaatatattgtggtgtaaacaaattgacgcttagacaacttaataacacattgcggacgtttttaatgtactggggtggttttaaccgtacatcactagtgatctagtaacatagatgacaccgcgcgcgataatttatcctagtttgcgcgctatattttgttttctatcgcgtattaaatgtataattgcgggactctaatcataaaaacccatctcataaataacgtcatgcattacatgttaattattacatgcttaacgtaattcaacagaaattatatgataatcatcgcaagaccggcaacaggattcaatcttaagaaactttattgccaaatgtttgaacgatcacgcaaattcagatctgagtaactggtctaacaggtctaggaggagcaggaagctcgaaatctctttgccagaatccaacatcatgccatccaccgtgcttgtatccagcagctctaagagttcctctagcagtgtatccaagagcctcatgaagtctaacagaaggatcgttagggagtccgataacagcaacaacagacttgaatccctgagcttccatagacttgagaaggtgagtgtaaagggtagatccaagtccaagtctctgatgtctgtgtgaaacgtaaacggtagactcaacagtccaatcgtaagcgtttctagccttccaaggtccagcgtaagcgattccagcaacaacaccctcaacctcagcaacaagccaagggtatctatcttggagtctctcaagatcatcgatccactcttgaggagtttgaggctcagttctgaagttaacggtagaagtctcgatgtagtggttcacgatatcacaaacagcagccatatcagcagcagtagcaggtctgatttcaacaggacgcctctcagggctcatatttaattcagtcccccgtgttctctccaaatgaaatgaacttccttatatagaggaagggtcttgcgaaggatagtgggattgtgcgtcatcccttacgtcagtggagatatcacatcaatccacttgctttgaagacgtggttggaacgtcttctttttccacgatgctcctcgtgggtgggggtccatctttgggaccactgtcggcagaggcatcttcaacgatggcctttcctttatcgcaatgatggcatttgtaggagccaccttccttttccactatcttcacaataaagtgacagatagctgggcaatggaatccgaggaggtttccggatattaccctttgttgaaaagtctcaattgccctttggtcttctgagactgtatctttgatatttttggagtagacaagtgtgtcgtgctccaccatgttgacgaagattttcttcttgtcattgagtcgtaagagactctgtatgaactgttcgccagtctttacggcgagttctgttaggtcctctatttgaatctttgactccatgggatccgcggccgccctgcaggctagaatctaattattctattcagactaaattagtataagtatttttttaatcaataaataataattaataatttattagtaggagtgattgaatttataatatattttttttaatcatttaaagaatcttatatctttaaattgacaagagttttaaatggggagagtgttatcatatgacaagtaggattaatgtgttatagtttcacatgcattacgataagttgtgaaagataacattattatatataacaatgacaatcactagcgatcgagtagtgagagtcgtcttattacactttcttccttcgatctgtcacatggcggcggcccttatcacttagaagcgtggtgcttcatgtagtagaagtttccgaaaagcatgaggagggtaaccatgtaaacaacgaggagttgagcaatgaacttagggtaaggagaagaagagtagaggaggtaaacagcctggagaaggttcatgaagaactggaacatttgcatctgggtaaggtatcttccccaccaaaggtactttctcttggtcttttcgtccttaggaagaacagcagccatgaagtagtaggtgtacatgcacacatgaacccaagagttgagagcagcagagaagtaagcatctccacctggagcagcataagtgatcatccaccagattccagagatagatccgtggtggtaaacatggaggaaggaaacctggttaacgtttcccttgagaagcatgatgaaggtgtccatgaactcgtagatcttggacacgtagaagatccagatcaccttagccatctcggtttgagcagggttgtaagcgtttccccagaaggagtacttgttcacgtaagcctcgtaaacgagcttgaggcacatgtaaaggctgagtccgataaggaaaacgttgtgagcgagcataagagccttgagaaggaaaggatcctgtcccttaacggttctagggaacactttacggtaaacgagtccagaaccaacgatagcgaagtaagcgaggagagaaaggataagaggggtaggagattcaacgagagggagatccttagtagcagaagagataggcttgagtccccatccaatagagtcggtagcagagaagatagcaggagcaacaacagcatcgatagcagcgtactgctcttgagccatagcaacgagaggttgagcaaattccatggtatggtaattgtaaatgtaattgtaatgttgtttgttgtttgttgttgttggtaattgttgtaaaatgctctgtttgtgtcggaaaataatggaggaagctatgagatgtatttgtatggatcctcttttgtggtccgttacgttttacaaagcatgcatttagacatgtgtatactcaaactcatgcatccatacacattgtaataaagtagtagtccactgaaagttgccaaaatagcaaaatagtacattgcagaaatatatatactaaattcatatatttcgatggaaaatttcggttttccacttaaaataaaatgtacgtataaacttagtcttcttttaacgccaaaaaaaagtctacaaatttctgtctttaatactacattatttttgaattgtgctaaactatgattacatgtgcattaaaatttgagggaatgtgtgttcttagatctgattggcataccctctgactaattatgggatcatgagtatttctcgggaatgtgtttattcgcaagtctattctctaacctcagtaaataatgagtggaagtttagttaaggccaaatagtctaaaatatattatttgtagttttgtacacagccaggattgaatcttaagagactctttaagtctaaaattacaatcagatcctagaccactttctatttgcatgaacgtaaccggatactgattttttaaatgttttctttggttcaaaatcgccactatctttgacaaaaacattctcgaataggattcaaacctaagagcctttcaaattcgttcttaattatgtcatcatctttagttctgctcccatctctcatcggtctcaagaaccactcctagtcatttaagtactacgttttatacacattacatatacatacatttacacaactaggaattgagtagggaacaaagtttcaactttcaactaatagggtaagccttctggtacatggaaaccaaccaaccaatctactagcctgcaggactattttcagaagaagttcccaatagtagtccaaaatttttgtaacgaagggagcataatagttacatgcaaaggaaaactgccattctttagaggggatgcttgtttaagaacaaaaaatatatcactttcttttgttccaagtcattgcgtatttttttaaaaatatttgttccttcgtatatttcgagcttcaatcactttatggttctttgtattctggctttgctgtaaatcgtagctaaccttcttcctagcagaaattattaatacttgggatatttttttagaatcaagtaaattacatattaccaccacatcgagctgcttttaaattcatattacagccatataggcttgattcattttgcaaaatttccaggatattgacaacgttaacttaataatatcttgaaatattaaagctattatgattaggggtgcaaatggaccgagttggttcggtttatatcaaaatcaaaccaaaccaactatatcggtttggattggttcggttttgccgggttttcagcattttctggttttttttttgttagatgaatattattttaatcttactttgtcaaatttttgataagtaaatatatgtgttagtaaaaattaattttttttacaaacatatgatctattaaaatattcttataggagaattttcttaataacacatgatatttatttattttagtcgtttgactaatttttcgttgatgtacactttcaaagttaaccaaatttagtaattaagtataaaaatcaatatgatacctaaataatgatatgttctatttaattttaaattatcgaaatttcacttcaaattcgaaaaagatatataagaattttgatagattttgacatatgaatatggaagaacaaagagattgacgcattttagtaacacttgataagaaagtgatcgtacaaccaattatttaaagttaataaaaatggagcacttcatatttaacgaaatattacatgccagaagagtcgcaaatatttctagatattttttaaagaaaattctataaaaagtcttaaaggcatatatataaaaactatatatttatattttggtttggttcgaatttgttttactcaataccaaactaaattagaccaaatataattgggatttttaatcgagatagaacccacacgagcatgtgctttccatttaattttaaaaaccaagaaacatacatacataacattccatcagcctctctctctttttattacggttaatgacttaaaacacatcttattatcccatccttaacacctagcagtgtctttatacgatctcatcgatcaccacttcaaaaccatgcagactgctgctgcccctggagctggcatcggctaggctgggtgccgcactgtcccggaaggtccctagcgacttgtttagattgatgggaccacctctcaacttcctgctgctgtccctgctgctggatgtcctgcctcatctggccgattgcacgctccagtcccctgcatgtgcactcgctcctcaattgcttaagatcatcgcagcagctatcgaagtgctggctctgttgccctcctccacggccttggttgtagtagtagctgcggcggcccttctggactttttcccacaggaaccgccgaataattcgatagaaccacacgagcatgtgctttcatttattttaaaaaccaagaaacatacataacatttcatcagcctctctctctctctctctctctctctctctctctctctctctctctctctctttattacagctgttacactaacttaaaacacattcatctcattattattattattatccatccttaacacctagcagtgtctttgtacgatctcataatcgatcaccccttcattacttctcagcagctccaactccgcagttgttgatgttacggaacatgagaacaccgttatcaccgtcaacgtattggcaagacctgaaagacttccaaagtgacttccacatgttctcgtcgctagacctgtagtgctttcccataactttcttgatagcctcagaagcaggtctagcgttgtagaatgggatcctagaacagtagtggtgaagcacatgagtctcgatgatatcatggaagatgtgaggtccgatgaatccgaactttctatcgatagtagcagcagcacccttagcgaaagtccattcctcagcgttgtaatgaggcatagtaggatcagtgtgctgaaggaatgtgatgaaaacgagccagtggttaacccagatgtaaggaacgaaccagttgatgaaaagggaccatcctccgaatttcttgtaccaaagagtaagaacgattccctgggtgaggattccaagatcagaaaggaagatgtagagagcatctctttgctcgaaaagtggagaggtaagccagaagtggttccatttccaagaaggaacatcagggtaaggttgtcctgtaacgttaacgaagaggtaagcgatccatcctccaagttgttgaacaagaagctcgtaaagggttctaagtggagaatcctcagagtactcagcgaggttaccgaagaagttcctagacttcttgaattcctctttggtggcaggaacgaaaaccatatctctggtcatgtgtccagtagccttatggtgctttccatgagagtacttccagctgaagtaaggaaccataaggtaagagtgaagggtccatccaacgaaatcgttcacgattccgtaatcagagaaagcttgatgtccacactcatgagcgagaacccagattccggttccgaaaagtccttgaacgtaagtgtaaagggcccagaaagtgaacttgatgatgctgttagaggtgtaagagatgaggagagggtaaaggatcttatgggtaaggtatccggtggtaagcatgcagaagatatctctgaacacgtagtagagagaggtagccaatcttctctcgtaacactcatgagggatagctccaaggatgtccttgatggtgaaatcaggaacagagaacacgtttccgttggtatcgatagcaacttttggaacctcttgctcggtgttgctagaagatcctctgttcttaggatcagatccagtaacggtaacagcgctcatggtatggtaattgtaaatgtaattgtaatgttgtttgttgtttgttgttgttggtaattgttgtaaaatttttggtggtgattggttctttaaggtgtgagagtgagttgtgagttgtgtggtgggtttggtgagattggggatggtgggtttatatagtggagactgaggaatggggtcgtgagtgttaactttgcatgggctacacgtgggttcttttgggcttacacgtagtattattcatgcaaatgcagccaatacatatacggtattttaataatgtgtgggaatacaatatgccgagtattttactaattttggcaatgacaagtgtacatttggattatcttacttggcctctcttgctttaatttggattatttttattctcttaccttggccgttcatattcacatccctaaaggcaagacagaattgaatggtggccaaaaattaaaacgatggatatgacctacatagtgtaggatcaattaacgtcgaaggaaaatactgattctgcccgttcgactcagatcttccaaggcctcgtctccgagtccgctgcttctcgccgcgccgatcacttctccgccgccaacaaggcttgtagttaataggaatcattcagggattgtgattccgggcagtagtaattaataatatagtattagtatagataatatgtttcgtttgggatctttggaacgttgctctgttccttgttgttcattttaaagcttttgagggatagttgcagaactgttcggtgatgcttcatcctctcaagaactagatttgggtaaagaaacatccatgcatggatatggaatgttgttcttccgattggagattattttataaaatttaaaattcatgatttaaaaaaacacataaaaaccacaaaattcatgatttattgacaatacgatacaaaattagcaccaccggctactggctcattacacatttccccttcccctcattctcactttgtggctttattattattattattacatatattttaccgttattatttcacgtcacataagcttgtcattactcagccttagatctaggccttcttccaagagcgtacatatgtctgagggtagaagcaaggttagaccagatagtagggtagtgcttgtactcgattcctctagcctcaagctcagccttaacaagaggagcaagtctagggtagaatccatggtgaactctagggaacaagtgatgctcaatttggtagttgagtccaccgttaagagtagcaagaagaggtcctccaacgttagaagaagtctcagcttgtctcttaaggaagctagcacctctagtcatagaagtgatagatccatcaggtccaacagaagcaacaccctcgaagttgtgggagatgaagaagaagaaagcgaggtagaaagatccagtcataacagtagcagcgatacacacagcagtatgaacagaaggagcaaggtaaagaggcaaagcaacgaatctagcccagaaggtaagcttgagaagcaaagaaggcataaagaggtatccagcaagcttagagataggctcaccctcccaacgccacataacaagctcagagatgtcgaggaacaaaagcttgaaagcgtacatagtctcaccaggcaaaaggtaaagatgctgaagccaatgcataggtgaccaagcatcagtaggcttgagtctaagagcaccgtgagccttttgatcaggatccttatcaacatcgttagtgtggaggtggtgcataacaacatgctcttgaagccaaaggatcatagatcctccgatccaatcctgacaaagtccaagagcaaggttaacagaagcagacttagacaaagcaccatggttagcatcatgctggatgttaagaccgataagagcgaaaagccatccaagaacgatagaagggagaagtctctttccagcgtaaagcatgtaagcctcaagagcgatagcagatccaaggataagtccagccttaacccagtaagaagcaggagcgaatccagaagaaacagaaggcaccatcttagcgatcctagcacaaagttgaaggtatccctcatcagcagcaacaggttcctcagtagaagcaagagatccaacgtggaatctagacattctagacttaggccaagcccttctatggtattccatgaaagcctcagtagcatctcttcctccgaacaaagaaacgaaatgagcaccaccaggatgctcagatctgaaagccttagcatcgtaaacagaatctccaacgatggtgagatcaggtctatcagcaacatcctttctggtgaaagcagaagagtcagtaacaccagcatgaacaccagtagaagctcccatttgcttagcagcgctaggtggcatggtatggtaattgtaaatgtaattgtaatgttgtttgttgtttgttgttgttggtaattgttgtaaaagtgggtatcttttggatggataagcaagtagtgatgatgttctaggtgaagtgatgggggtgttttatagcgggagatggtgaaatggatggtcgccacataagaaatggaggggaagggttcttgcgccattcttcagtttgcatggatgcatgggtttcattttgtaacacgtaataaggacaatgaagtgcaggtgtctctcaagtttcagaggggatatgtggacagaagaagaacggcgatgatattgatggaaatggccatctagtgtgaatctattcggttgataatactagtgcattttggccgttaatcccttcaattaactgcacaaacttcagttgagtattgattatttgattataggttctgtaaacacaataccaagtttatttagaggggagacatacaaatagtttcgatataaataatagagtggttaaacttagttattaaaactatatataaagtctaaaagttaaattatttttttaattgcaaatatataaagtctaaaggggttacattatttcttaagagatgtaactctgttggaatctgacttaatccgtctcatcactctggtttccagttctaatctaatgaattgttttctgccaaagaatttgaagcaagaagtaaattgatcaatgccgtcaacccacaccaaaccgtcaacccactaccatcgccgcggagacccccaaactcaacctccacccatcggtaagaagcacagggcagcccgcaccaccaccaatttggcgtgcatgacacctagggacttggcacgggaggcggcgcacgtggatgcaaatgacgggatatcagatgacaggaaacgacgttgagagaccatacgatgtagaatatgagctcaccatcaacgagaaactaggaaaatcacaaaaaaaacaactctcgtaattgtacgagtggcacagatgggtctgcctcaacatatctctaatacggcgaagcctgcccaacacgtagttgccggaatccggtgtggagctcacgactctgaaagataggcgcttcctgtttcgtttcgctcacccactggacgtccgtcatgtgatggatttcggtcattggtttgctgacaaccacattctgaagctccatgagatgagtcttcacaataggtcctgctcaataccgtggagttatggttgcaagtccataacttgccgttcgaatattttgcggagccagtcggacgggaattggcgagctcggctgacacctataaaggccatgacaagaagaaccaaaagttcttccctaatgctttcatgaggcttcgggtcgttatggatgtcggaaaacccctcttgaaggaacgagacgttattatgcatgacggtaagactattacttgtcagtataagtatgaaagattacctgtcttctgctttgtttgtggattgattggacacgttgaaaaaaaatgtgcacttcgatttcaatactcagagatcgacttcccttttctctaggagtattcgatcaaggcattaacatggaaggaagctcaagctctaaaggcttcacaatggaacctgaaaaatttcaacaagcctaaactgaaatcgaagtcaaatcacccaaccgggagctctaaatcagcaaacactcctcctccacagtatccaatcatcgtgcacgatgctccaggtattgcaagccaggtattgcaagctaggagtaggatagagaccttaaacgtcgttggtgtgaagagtcatcttcagacctaatggagatagatgtagacggcggcacgaagactctgaaacaccagaaaggctagtccaggataaggatctgctatcccaactgacctctcgttagtcccaaggcctctcaactagagcaggaggaaggatggtcacaagactaggataatgatgtttccaatatgaacctgaatgtccatagctaatttttttagtcttgcttctgcactttttgtttattatgttctggtgactatgttatttacccttgtccgtatgcttgagagaatcagtattttccttcgacgttaattgatcctacactatgtaggtcatatccatcgttttaatttttggccaccattcaattctgtcttgcctttagggatgtgaatatgaacggccaaggtaagagaataaaaataatccaaattaaagcaagagaggccaagtaagataatccaaatgtacacttgtcattgccaaaattagtaaaatactcggcatattgtattcccacacattattaaaataccgtatatgtattggctgcatttgcatgaataatactacgtgtaagcccaaaagaacccacgtgtagcccatgcaaagttaacactcacgaccccattcctcagtctccactatataaacccaccatccccaatctcaccaaacccaccacacaactcacaactcactctcacaccttaaagaaccaatcaccaccaaaaattttacaacaattaccaacaacaacaaacaacaaacaacattacaattacatttacaattaccataccatgtctaaggttaccgtgtctggatctgagatccttgagggatctactaagaccgttaggcgttctggaaacgttgcatctttcaagcagcaaaagaccgctatcgataccttcggaaacgttttcaaggtgccagattacaccatcaaggatatccttgacgctatccctaagcactgttacgagagatctctcgtgaagtctatgtcttacgtggtgagagatatcgtggctatctctgctatcgcttacgttggacttacctacatccctcttctccctaacgaattccttagattcgctgcttggtctgcttacgtgttctctatctcttgtttcggattcggaatctggatccttggacatgagtgtggacattctgctttctctaactacggatgggttaacgataccgttggatgggttctccactctcttgttatggttccttacttcagctggaagttctctcatgctaagcaccataaggctactggacacatgaccagagatatggttttcgttccttacaccgccgaggaattcaaagagaagcaccaagttaccagccttcacgatatcgctgaggaaactcctatctactctgttttcgctctcttgttccaacagcttggaggactttctctttaccttgctactaacgctactggacaaccttaccctggtgtttctaagttcttcaagtctcactactggccttctagccctgttttcgataagaaggactactggtacatcgttctttctgatcttggaatccttgctaccctcacttctgtttacaccgcttacaaggttttcggattctggcctactttcatcacatggttctgtccttggatccttgttaaccactggcttgttttcgttaccttccttcagcacaccgattcttctatgcctcattacgatgctcaagagtggactttcgctaagggtgctgctgctactatcgatagagagttcggaatcctcggaatcatcttccatgacatcatcgagactcatgtgctccatcactacgtttcaaggatcccattctaccatgctagagaagctaccgagtgcatcaagaaagttatgggagagcactacagacacaccgatgagaacatgtgggttagcctttggaaaacttggagatcttgccagttcgttgagaaccatgatggtgtgtacatgttccgtaactgcaacaacgttggagtgaagcctaaggatacctgatgaaggggtgatcgattatgagatcgtacaaagacactgctaggtgttaaggatggataataataataataatgagatgaatgtgttttaagttagtgtaacagctgtaataaagagagagagagagagagagagagagagagagagagagagagagagagagaggctgatgaaatgttatgtatgtttcttggtttttaaaataaatgaaagcacatgctcgtgtggttctatcgaattattcggcggttcctgtgggaaaaagtccagaagggcggcggcagctactactacaaccaaggccgtggaggagggcaacagagccagcacttcgatagctgctgcgatgatcttaagcaattgaggagcgagtgcacatgcaggggactggagcgtgcaatcggccagatgaggcaggacatccagcagcagggacagcagcaggaagttgagaggtggtcccatcaatctaaacaagtcgctagggaccttccgggacagtgcggcacccagcctagccgatgccagctccaggggcagcagcagtctgcatggttttgaagtggtgatcgatgagatcgtataaagacactgctaggtgttaaggatgggataataagatgtgttttaagtcattaaccgtaataaaaagagagagaggctgatggaatgttatgtatgtatgtttcttggtttttaaaattaaatggaaagcacatgctcgtgtgggttctatcactattttcagaagaagttcccaatagtagtccaaaatttttgtaacgaagggagcataatagttacatgcaaaggaaaactgccattctttagaggggatgcttgtttaagaacaaaaaatatatcactttcttttgttccaagtcattgcgtatttttttaaaaatatttgttccttcgtatatttcgagcttcaatcactttatggttctttgtattctggctttgctgtaaatcgtagctaaccttcttcctagcagaaattattaatacttgggatatttttttagaatcaagtaaattacatattaccaccacatcgagctgcttttaaattcatattacagccatataggcttgattcattttgcaaaatttccaggatattgacaacgttaacttaataatatcttgaaatattaaagctattatgattaggggtgcaaatggaccgagttggttcggtttatatcaaaatcaaaccaaaccaactatatcggtttggattggttcggttttgccgggttttcagcattttctggttttttttttgttagatgaatattattttaatcttactttgtcaaatttttgataagtaaatatatgtgttagtaaaaattaattttttttacaaacatatgatctattaaaatattcttataggagaattttcttaataacacatgatatttatttattttagtcgtttgactaatttttcgttgatgtacactttcaaagttaaccaaatttagtaattaagtataaaaatcaatatgatacctaaataatgatatgttctatttaattttaaattatcgaaatttcacttcaaattcgaaaaagatatataagaattttgatagattttgacatatgaatatggaagaacaaagagattgacgcattttagtaacacttgataagaaagtgatcgtacaaccaattatttaaagttaataaaaatggagcacttcatatttaacgaaatattacatgccagaagagtcgcaaatatttctagatattttttaaagaaaattctataaaaagtcttaaaggcatatatataaaaactatatatttatattttggtttggttcgaatttgttttactcaataccaaactaaattagaccaaatataattgggatttttaatcgaccgatctagtaacatagatgacaccgcgcgcgataatttatcctagtttgcgcgctatattttgttttctatcgcgtattaaatgtataattgcgggactctaatcataaaaacccatctcataaataacgtcatgcattacatgttaattattacgtgcttaacgtaattcaacagaaattatatgataatcatcgcaagaccggcaacaggattcaatcttaagaaactttattgccaaatgtttgaacgatctcattactgcattttcttctcaggagcatgggcaacgttatcaaggttagcgaaagtatcagccatagcctcgaagtatcctctaacatcgtagtgaagtccgtgcttctcgaaaagctgcttaactctaggagcgatcttagggtgtctgaattgaggcatagaagggtaaaggtggtgctcgatctggtagttaaggtaagacatccaccaatcacaccaccaagatggagaacagttagtagtgtggttagcagcgtactcaacccaagtagcatgctcgttaggctcaacaacagggaggtgagtatgagaaacagcgaagttgcagaagatgtacatagctccaagctgaacgtaaagaaggtaacaagcgagaacgtatccagcaccgtagttagcagcaaggtatccaacaagtccgtatctgattccgagcatagcaagctcatcgtagtgcttagtcctgagcatgtgtctaggatgaaggtaaagctgccatccaagagcaacaagaagagtggtaacaggagcgaaaagcttagcttgcatagaaagccaagccttcatagcaggagacttaaccttagcagcgattctctcatggaaagcaacgagaggaagggtatcaagatcaacatcgtgctgaagcttttgaggagtagcatggtgcttgttatgctggttacgccaccaagcaccagacattccacatccaagtccgtaacaagcaacttggatagctctgtcgaaagcaatgtttccagtgagagagtaatgtccaccctcatgcataagccatccacatcttccctgaacaactccaagcatagcgattccagcgaaagtgtatccatgccagataagagcagcaccagcaacatgcatagcgataacctcagcaagtctgtaagcaacatgaggaagagaaggctcgaacattccctcagcctcaagttgcttggtgaactcttggaaatcagcgataagatcagcccttcttggagagtatcccttgtgaacaggacgagaaggaagagacttaagcatcttgtcagccttagcagatctaacatggaactgcttgtaagcatcggtagcatcagttccaacttggtaagcaatgatctttccaccagggtgtctcttaacgaagttggtaacatcgtaagccctatctccgataacaagctctttcttgtcgtgctcttgaggagtatcaacttcgtgaagttgagcagaaggaggagcagcataagagtaagagtcccttggaggcatggtatggtaattgtaaatgtaattgtaatgttgtttgttgtttgttgttgttggtaattgttgtaaaagatcctcgtgtatgtttttaatcttgtttgtatcgatgagttttggtttgagtaaagagtgaagcggatgagttaatttataggctataaaggagatttgcatggcgatcacgtgtaataatgcatgcacgcatgtgattgtatgtgtgtgctgtgagagagaagctcttaggtgtttgaagggagtgacaagtggcgaagaaaaacaattctccgcggctgcatgctatgtgtaacgtgtagctaatgttctggcatggcatcttatgaacgattctttttaaaaacaaggtaaaaacttaacttcataaaattaaaaaaaaaaacgtttactaagttggtttaaaaggggatgagactagaatctaattattctattcagactaaattagtataagtatttttttaatcaataaataataattaataatttattagtaggagtgattgaatttataatatattttttttaatcatttaaagaatcttatatctttaaattgacaagagttttaaatggggagagtgttatcatatgacaagtaggattaatgtgttatagtttcacatgcattacgataagttgtgaaagataacattattatatataacaatgacaatcactagcgatcgagtagtgagagtcgtcttattacactttcttccttcgatctgtcacatggcggcggcccggcgcgccgcgcgccttatcactgcttcttagcacccttagacttgtacctcttacggtagaagttggcgaagagaacgaacatgttcaccataacccagagttgaaggtaaggaagccagaaagcggtattctgaacgtaagcggtgtagatagagtgagaagcacagatacagaactgaagcatctggatctgggtgatgtacttcttccagaaacagttaactccaagagcagcaagtccgtagtaagagtacatgatcacgtgcacgaaggtgttaacagaagatccgaagtagcaatctccaacaggctcaagcttcataacaacgaaccatgaccagatgagaagagtgtggtggtagatgtgaaggaaagaaagctggtcgaacttcttcctcatcaccatgaagaaggtgtcgagaagctcaacgtacttgttgttgtagtgaagccagataacctgagagattccccaagagttagcagtcatatcagggatgtttccccaaaccttaagtccctgagccctatgagaagtaacgaaaaggtagatgcagtagctgttgaagaaggtctggtagaagttgtaaacgagcatagcgttcttgagtccgaaaggttgagatctgttctgcatgatacgctttccgaagtagatgaagaggaggtatccaatagttccgatagtaggtccccagtactcaacctgcatgaagtaagcaggaactttctcagaagctgggatatcagggttagccacattgtaggtaacgtatccaagagttccagcaagagcagcagggatagcgatagaggccatggtatggtaattgtaaatgtaattgtaatgttgtttgttgtttgttgttgttggtaattgttgtaaaatgctctgtttgtgtcggaaaataatggaggaagctatgagatgtatttgtatggatcctcttttgtggtccgttacgttttacaaagcatgcatttagacatgtgtatactcaaactcatgcatccatacacattgtaataaagtagtagtccactgaaagttgccaaaatagcaaaatagtacattgcagaaatatatatactaaattcatatatttcgatggaaaatttcggttttccacttaaaataaaatgtacgtataaacttagtcttcttttaacgccaaaaaaaagtctacaaatttctgtctttaatactacattatttttgaattgtgctaaactatgattacatgtgcattaaaatttgagggaatgtgtgttcttagatctgattggcataccctctgactaattatgggatcatgagtatttctcgggaatgtgtttattcgcaagtctattctctaacctcagtaaataatgagtggaagtttagttaaggccaaatagtctaaaatatattatttgtagttttgtacacagccaggattgaatcttaagagactctttaagtctaaaattacaatcagatcctagaccactttctatttgcatgaacgtaaccggatactgattttttaaatgttttctttggttcaaaatcgccactatctttgacaaaaacattctcgaataggattcaaacctaagagcctttcaaattcgttcttaattatgtcatcatctttagttctgctcccatctctcatcggtctcaagaaccactcctagtcatttaagtactacgttttatacacattacatatacatacatttacacaactaggaattgagtagggaacaaagtttcaactttcaactaatagggtaagccttctggtacatggaaaccaaccaaccaatctactagggtaccctcaagcatacggacaagggtaaataacatagtcaccagaacataataaacaaaaagtgcagaagcaagactaaaaaaattagctatggacattcaggttcatattggaaacatcattatcctagtcttgtgaccatccttcctcctgctctagttgagaggccttgggactaacgagaggtcagttgggatagcagatccttatcctggactagcctttctggtgtttcagagtcttcgtgccgccgtctacatctatctccattaggtctgaagatgactcttcacaccaacgacgtttaaggtctctatcctactcctagcttgcaatacctggcttgcaatacctggagcatcgtgcacgatgattggatactgtggaggaggagtgtttgctgatttagagctcccggttgggtgatttgacttcgatttcagtttaggcttgttgaaatttttcaggttccattgtgaagcctttagagcttgagcttccttccatgttaatgccttgatcgaatactcctagagaaaagggaagtcgatctctgagtattgaaatcgaagtgcacattttttttcaacgtgtccaatcaatccacaaacaaagcagaagacaggtaatctttcatacttatactgacaagtaatagtcttaccgtcatgcataataacgtctcgttccttcaagaggggttttccgacatccataacgacccgaagcctcatgaaagcattagggaagaacttttggttcttcttgtcatggcctttataggtgtcagccgagctcgccaattcccgtccgactggctccgcaaaatattcgaacggcaagttatggacttgcaaccataactccacggtattgagcaggacctattgtgaagactcatctcatggagcttcagaatgtggttgtcagcaaaccaatgaccgaaatccatcacatgacggacgtccagtgggtgagcgaaacgaaacaggaagcgcctatctttcagagtcgtgagctccacaccggattccggcaactacgtgttgggcaggcttcgccgtattagagatatgttgaggcagacccatctgtgccactcgtacaattacgagagttgttttttttgtgattttcctagtttctcgttgatggtgagctcatattctacatcgtatggtctctcaacgtcgtttcctgtcatctgatatcccgtcatttgcatccacgtgcgccgcctcccgtgccaagtccctaggtgtcatgcacgccaaattggtggtggtgcgggctgccctgtgcttcttaccgatgggtggaggttgagtttgggggtctccgcggcgatggtagtgggttgacggtttggtgtgggttgacggcattgatcaatttacttcttgcttcaaattctttggcagaaaacaattcattagattagaactggaaaccagagtgatgagacggattaagtcagattccaacagagttacatctcttaagaaataatgtaacccctttagactttatatatttgcaattaaaaaaataatttaacttttagactttatatatagttttaataactaagtttaaccactctattatttatatcgaaactatttgtatgtctcccctctaaataaacttggtattgtgtttacagaacctataatcaaataatcaatactcaactgaagtttgtgcagttaattgaagggattaacggccaaaatgcactagtattatcaaccgaatagattcacactagatggccatttccatcaatatcatcgccgttcttcttctgtccacatatcccctctgaaacttgagagacacctgcacttcattgtccttattacgtgttacaaaatgaaacccatgcatccatgcaaactgaagaatggcgcaagaacccttcccctccatttcttatgtggcgaccatccatttcaccatctcccgctataaaacacccccatcacttcacctagaacatcatcactacttgcttatccatccaaaagatacccacttaattaattttacaacaattaccaacaacaacaaacaacaaacaacattacaattacatttacaattaccataccatgtgccctcctaagactgatggaagatcttctcctagatctccacttaccaggtctaaatcttctgctgaggctcttgatgctaaggatgcttctactgctcctgttgatcttaagactcttgagcctcatgagcttgctgctactttcgagactagatgggttagagttgaggacgttgagtacgatgtgactaacttcaagcaccctggtggatctgtgatcttctacatgcttgctaacactggtgctgatgctactgaggctttcaaagaattccacatgcgttctctcaaggcttggaagatgcttagagctttgccttctagacctgctgagatcaagagatctgagtctgaggatgctcctatgcttgaggatttcgctagatggcgtgctgagcttgagagagatggattcttcaagccttctatcacccatgtggcttacagacttctcgagcttcttgctacattcgctcttggaactgctcttatgtacgctggataccctatcattgcttctgttgtttacggtgctttcttcggagctagatgtggatgggttcaacatgagggtggacataactctcttaccggatctgtttacgtggacaagagacttcaggctatgacttgtggattcggactttctacttctggtgagatgtggaaccagatgcataacaagcaccatgctacccctcaaaaggttagacacgatatggatcttgataccactcctgctgtggctttcttcaacactgctgttgaggataacagacctagaggattctctagagcttgggctagacttcaagcttggactttcgttcctgttacctctggacttcttgttcaagctttctggatctacgttctccaccctagacaagttctccgtaagaagaactacgaagaggcttcttggatgctcgtttctcatgttgttagaaccgctgttatcaagcttgctactggatactcttggcctgttgcttactggtggttcactttcggaaactggatcgcttacatgtaccttttcgctcacttctctacttctcatactcacctccctgttgttccatctgataagcacctttcttgggttaactacgctgttgatcacaccgttgatatcgatccttctagaggatacgtgaactggcttatgggataccttaactgtcaggttatccaccacctcttccctgatatgcctcaattcagacagcctgaggttagcagaagattcgttcctttcgctaagaagtggggactcaactacaaggtgctctcttactacggtgcttggaaggctactttctctaaccttgataaggtgggacagcactactacgttaacggaaaggctgagaaggctcactaatgattaattaacaagcttatgtgacgtgaaataataacggtaaaatatatgtaataataataataataaagccacaaagtgagaatgaggggaaggggaaatgtgtaatgagccagtagccggtggtgctaattttgtatcgtattgtcaataaatcatgaattttgtggtttttatgtgtttttttaaatcatgaattttaaattttataaaataatctccaatcggaagaacaacattccatatccatgcatggatgtttctttacccaaatctagttcttgagaggatgaagcatcaccgaacagttctgcaactatccctcaaaagctttaaaatgaacaacaaggaacagagcaacgttccaaagatcccaaacgaaacatattatctatactaatactatattattaattactactgcccggaatcacaatccctgaatgattcctattaactacaagccttgttggcggcggagaagtgatcggcgcggcgagaagcagcggactcggagacgaggccttggaagatctgagtcgaacgggcggtaccgcggccgcaagctttccgcggggcgcccgttttacaacgtcgtgactgggagatccactagcagattgtcgtttcccgccttcagtttaaactatcagtgtttgaaggacagacccacccaagaacacaccagtcattcagatgcagcctatctccgtgccggctattccagctgatgagttgaaggatataactgataactatggttccaagtccttgattggtgagggctcttatggaagagtgttttacggtgttcttagaagcggcaaggcagctgccattaagaagctggattctagtaagcagcctgatcaagagtttctcgcacaggtacaaatgctacttaagtaaatcaaaccgttaaagttgagttgctgcttagttactgatgtaaataatgttaattaggtatcaatggtttcgagattgagacaagacaatgttgttgcacttctgggatattgcgttgatggcccactccgtgttcttgcttatgagtttgctcctaatggatctcttcatgatattcttcatggtaagttattaagtctaaaacattgattcggtacgacttgtagatgtgaagctattaactaatgaaatgtggtgagtttgttgggtgtaggtaggaaaggagtgaaaggagcacagccaggacctgttctgtcgtggaaccagagagttaaaattgctgttggtgcggctaggggactcgagtacttgcatgagaaggcgaaccctcatgttgtccaccgagacatcaaatccagcaatgtgcttttgtttgacgatgatgttgccaagattgctgacttcgatctgtctaaccaagcccctgacatggctgctcgccttcactcaactcgtgtgctgggaacctttggttatcacgctccagagtaagccctttacttgtttatttgaattgtttttgttcagactaatcaatgtggttacattcaacttgtgctcaaagacttttggttattattatcttatgttttgaggcactaagtccttccttggaataatctttgacattattttggattgcatctcttctaattgaccatactagagtcttaaacacaaacatttttgttttggttctgcattttcaggtatgcaatgacagggacattgagcacaaagagtgatgtctatagttttggagttgttctgctagagctcctcacaggtcgtaagccagttgatcataccttaccacgaggacagcagagtctcgttacatgggtaatgcttagtgcagctctgcttcttttttctggtttactcatattgagaagaaaagggaatgtgtctgcacaatcatgttgattttgtgagagattagataaactcattattaaatgaaaacgcgtttgtgtgtgtgtatcaggcaactcctaaactgagtgaagacaaggtgaagcaatgcgttgatgcaagactaaacggagaatatcctcccaaagctgttgccaaggtaaccttttgtcatagtgtcgttgtgtcagtagagaaggtttaccttaggacacgacttagaaactgcttctccatcacttccatcgttttcggttccttcttaatgtatccctgttgtaggcctagattgaaatacaagtctcttctaaggacaatagaacctaagcattgatgtatgatttttttgggagtctgattttggttttttctctcttatatgactccggtaatgatcagctggctgctgtagctgcgctatgtgtgcaatacgaagcagacttcaggccaaacatgagcatagtggtgaaggctcttcagcctctcctcaatcctcctcgctctgctcctcaaactcctcacaggaacaatccttattgatgtcctccaatctgatgccacgcttcttcatcatatcacttatttcatttgtttttgtttgaatccaatttgtgtaaattcgtgaaaataggctttttatttctcacaatagacatgaaagtctcacttccaaacctgaatggtgttgctctatttgtttatgttatttcatgcctgcgattgtaagtttctactaattatacaatatgcgaggaatggattattcataatatactcattgtgtttgtgcc

SEQ ID NO: 42 - DNA, 18 bp, synthetic construct
  misc_feature 1..18: note = Junction at 5' end of transgene
  source 1..18: mol_type = other DNA
tggaggtgttcaaacact

SEQ ID NO: 43 - DNA, 18 bp, synthetic construct
  misc_feature 1..18: note = Junction of 5' end of 4-transgene-insert on chr. A02.
  source 1..18: mol_type = other DNA
tggaggtgttcaaacact

SEQ ID NO: 44 - DNA, 18 bp, synthetic construct
  misc_feature 1..18: note = Junction of 3' end of 4-trangene-insert and chr. A02
  source 1..18: mol_type = other DNA
atagtattagtatacaga

SEQ ID NO: 45 - DNA, 18 bp, synthetic construct
  misc_feature 1..18: note = Junction of 5' end of 16-transgene insert in chr. A05
  source 1..18: mol_type = other DNA
ggctaaggtaacactgat

SEQ ID NO: 46 - DNA, 18 bp, synthetic construct
  misc_feature 1..18: note = Junction of 3' end of 16-transgene insert and chr. A05
  source 1..18: mol_type = other DNA
cagtgtttgaaggacaga

SEQ ID NO: 47 - DNA, 470 bp, synthetic construct
  misc_feature 1..470: note = 470 bp chimeric 5' junction of transgenic insert and Brassica chr. A02
  source 1..470: mol_type = other DNA
cattgagcagtgaacaccaaggataaatatttactgattagtgtgtgattgaatcaaagaaaggttagaatctggttttcatttagccattcaatctcgatgtaaaatcggttagattctggttgttgatacttgagaacttgaaatgttttgtaactgtgaattttgttttgaaaatagacaagtgaatctgtttggggttgtgtgaaaacgtgtgagcaattgttggaggtgttcaaacactgatagtttaaactgaaggcgggaaacgacaatctgctagtggatctcccagtcacgacgttgtaaaacgggcgccccgcggaaagcttgcggccgcggtaccgcccgttcgactcagatcttccaaggcctcgtctccgagtccgctgcttctcgccgcgccgatcacttctccgccgccaacaaggcttgtagttaataggaatcattcagggattgtgattccg

SEQ ID NO: 48 - DNA, 470 bp, synthetic construct
  misc_feature 1..470: note = 470 bp chimeric 3' junction of transgenic insert and Brassica chr. A02
  source 1..470: mol_type = other DNA
ttgaatggtggccaaaaattaaaacgatggatatgacctacatagtgtaggatcaattaacgtcgaaggaaaatactgattctgcccgttcgactcagatcttccaaggcctcgtctccgagtccgctgcttctcgccgcgccgatcacttctccgccgccaacaaggcttgtagttaataggaatcattcagggattgtgattccgggcagtagtaattaataatatagtattagtatacagaacctcttatttagctaaaagattatgttcttaatgttgataagaagtttgagaaacaaatataattgagcttctgattagttgatcgtaattggtcattaataattgtatctaaccagtgcagtataagagcgtataagagcatcttcaaaaagactttattttagagttaatcagtgcagtataagagcatctctaaaaaaactctaattatagagttttgcaaa

SEQ ID NO: 49 - DNA, 470 bp, synthetic construct
  misc_feature 1..470: note = 470 bp chimeric 5' junction of transgene insert and chr. A05
  source 1..470: mol_type = other DNA
cttgttccgcaacaccgttactgaactcttcgttcacttaaacagtttgtgtgtgtgagaaacagcgtaatgagctgctttggttgttgtggtggtgacgattttcgtcgagttgctgaaactggacccaagccagtgtacggcgcaggaggtactttaagcttataaccctttgtctatcctttggctagcggctaatgttgatgaacttttttattcaaccgttggctaaggtaacactgatagtttaaactgaaggcgggaaacgacaatctgctagtggatctcccagtcacgacgttgtaaaacgggcgccccgcggaaagcttgcggccgcggtaccgcccgttcgactcagatcttccaaggcctcgtctccgagtccgctgcttctcgccgcgccgatcacttctccgccgccaacaaggcttgtagttaataggaatcattcagggattgtgattccgggc

SEQ ID NO: 50 - DNA, 470 bp, synthetic construct
  misc_feature 1..470: note = 470 bp chimeric 3' junction of transgene insert and chr. A05
  source 1..470: mol_type = other DNA
ttattaattactactgcccggaatcacaatccctgaatgattcctattaactacaagccttgttggcggcggagaagtgatcggcgcggcgagaagcagcggactcggagacgaggccttggaagatctgagtcgaacgggcggtaccgcggccgcaagctttccgcggggcgcccgttttacaacgtcgtgactgggagatccactagcagattgtcgtttcccgccttcagttaaggacagacccacccaagaacacaccagtcattcagatgcagcctatctccgtgccggctattccagctgatgagttgaaggatataactgataactatggttccaagtccttgattggtgagggctcttatggaagagtgttttacggtgttcttagaagcggcaaggcagctgccattaagaagctggattctagtaagcagcctgatcaagagtttctcgcacaggtacaa

SEQ ID NO: 51 - DNA, 24 bp, synthetic construct
  misc_feature 1..24: note = Forward primer for amplicon diagnostic for NS-B50027-4
  source 1..24: mol_type = other DNA
aattgttggaggtgttcaaacact

SEQ ID NO: 52 - DNA, 24 bp, synthetic construct
  misc_feature 1..24: note = Reverse primer for amplicon diagnostic for NS-B50027-4
  source 1..24: mol_type = other DNA
cggaatcacaatccctgaatgatt

SEQ ID NO: 53 - DNA, 20 bp, synthetic construct
  misc_feature 1..20: note = Sense primer for detection of codon-optimized delta12-desaturase
  source 1..20: mol_type = other DNA
tggagctatccctcatgagt

SEQ ID NO: 54 - DNA, 21 bp, synthetic construct
  misc_feature 1..21: note = Antisense primer for detection of codon-optimized delta12-desaturase
  source 1..21: mol_type = other DNA
gatcctagaacagtagtggtg

SEQ ID NO: 55 - DNA, 21 bp, synthetic construct
  misc_feature 1..21: note = Sense primer for detecting codon-optimized delta15/omega3-desaturase
  source 1..21: mol_type = other DNA
gacgctatccctaagcactgt

SEQ ID NO: 56 - DNA, 20 bp, synthetic construct
  misc_feature 1..20: note = Antisense primer for detecting codon-optimized delta15/omega3-desaturase
  source 1..20: mol_type = other DNA
gtccactcttgagcatcgta

SEQ ID NO: 57 - DNA, 21 bp, synthetic construct
  misc_feature 1..21: note = Sense primer for detecting codon-optimized delta6-desaturase
  source 1..21: mol_type = other DNA
gagcaccttgtagttgagtcc

SEQ ID NO: 58 - DNA, 21 bp, synthetic construct
  misc_feature 1..21: note = Antisense primer for detecting codon-optimized delta6-desaturase
  source 1..21: mol_type = other DNA
agtctgaggatgctcctatgc

SEQ ID NO: 59 - DNA, 20 bp, synthetic construct
  misc_feature 1..20: note = Sense primer for detecting codon-optimized delta6-elongase
  source 1..20: mol_type = other DNA
tgttgctatggctcaagagc

SEQ ID NO: 60 - DNA, 20 bp, synthetic construct
  misc_feature 1..20: note = Antisense prmer for detecting codon-optimized delta6-elongase
  source 1..20: mol_type = other DNA
ctagcgtggtgcttcatgta

SEQ ID NO: 61 - DNA, 20 bp, synthetic construct
  misc_feature 1..20: note = Sense primer for detection codon-optimized delta5-desaturase
  source 1..20: mol_type = other DNA
gctaccgatgcttacaagca

SEQ ID NO: 62 - DNA, 20 bp, synthetic construct
  misc_feature 1..20: note = Antisense primer for detecting codon-optimized delta5-desaturase
  source 1..20: mol_type = other DNA
tagtgaagtccgtgcttctc

SEQ ID NO: 63 - DNA, 20 bp, synthetic construct
  misc_feature 1..20: note = Sense primer for detection of delta5-elongase
  source 1..20: mol_type = other DNA
tgctggaactcttggatacg

SEQ ID NO: 64 - DNA, 20 bp, synthetic construct
  misc_feature 1..20: note = Antisense primer for detection of codon-optimized delta5-elongase
  source 1..20: mol_type = other DNA
ctgggtgatgtacttcttcc

SEQ ID NO: 65 - DNA, 20 bp, synthetic construct
  misc_feature 1..20: note = Sense primer for detecting codon-optimized delta4-desaturase
  source 1..20: mol_type = other DNA
ggctttcagatctgagcatc

SEQ ID NO: 66 - DNA, 20 bp, synthetic construct
  misc_feature 1..20: note = Antisense primer for detecting codon-optimized delta4-desaturase
  source 1..20: mol_type = other DNA
ctcagccttaacaagaggag